European Patent Application EP 4 174 084 A1, published May 3, 2023. Title: Anti-RSV antibodies and pharmaceutical composition including the antibodies. Applicant: Mogam Institute for Biomedical Research. The sequence listing filed with the application follows.

SEQUENCE LISTING (530 sequences)

SEQ ID NO: 1 - protein, 6 aa, Artificial Sequence
  clone 8 heavy chain CDR1
SSYTMH

SEQ ID NO: 2 - protein, 17 aa, Artificial Sequence
  clone 8 heavy chain CDR2
SITGGSSYVDYSASVKG

SEQ ID NO: 3 - protein, 12 aa, Artificial Sequence
  clone 8 heavy chain CDR3
DDYGSGSYSNWF

SEQ ID NO: 4 - protein, 12 aa, Artificial Sequence
  clone 8 light chain CDR1
SSSDIGAGYDVH

SEQ ID NO: 5 - protein, 7 aa, Artificial Sequence
  clone 8 light chain CDR2
ANTNRPS

SEQ ID NO: 6 - protein, 8 aa, Artificial Sequence
  clone 8 light chain CDR3
QSYDRSLS

SEQ ID NO: 7 - protein, 12 aa, Artificial Sequence
  clone 9 light chain CDR1
SSSNIGAGYDVH

SEQ ID NO: 8 - protein, 6 aa, Artificial Sequence
  clone 13 heavy chain CDR1
TSYRMH

SEQ ID NO: 9 - protein, 17 aa, Artificial Sequence
  clone 13 heavy chain CDR2
SITGGGNYIEYADSVKG

SEQ ID NO: 10 - protein, 14 aa, Artificial Sequence
  clone 13 heavy chain CDR3
DMYGLGSYYSPNYF

SEQ ID NO: 11 - protein, 6 aa, Artificial Sequence
  clone 33 heavy chain CDR1
SSYGMN

SEQ ID NO: 12 - protein, 17 aa, Artificial Sequence
  clone 33 heavy chain CDR2
SISASSSFINYADSVRD

SEQ ID NO: 13 - protein, 11 aa, Artificial Sequence
  clone 33 light chain CDR1
SSNLGAGYDVH

SEQ ID NO: 14 - protein, 11 aa, Artificial Sequence
  clone 6m light chain CDR1
SSNIGAGYDVH

SEQ ID NO: 15 - protein, 7 aa, Artificial Sequence
  clone 6m light chain CDR2
GNSNRPS

SEQ ID NO: 16 - protein, 17 aa, Artificial Sequence
  clone 12m heavy chain CDR2
SITGGSSYLDYAHSVKG

SEQ ID NO: 17 - protein, 12 aa, Artificial Sequence
  clone 12m heavy chain CDR3
DDYGSGSYSNYF

SEQ ID NO: 18 - protein, 7 aa, Artificial Sequence
  clone 12m light chain CDR2
GSTNRPS

SEQ ID NO: 19 - protein, 123 aa, Artificial Sequence
  clone 8 heavy chain
EVQLVESGGGLIQPGGSLRLSCAGSGFTFSSYTMHWVRQAPGKGLEWVSSITGGSSYVDYSASVKGRFTISRDNAQSSLYLQMNSLRAEDTAVYYCARDDYGSGSYSNWFDPWGQGTLVTVSS

SEQ ID NO: 20 - protein, 111 aa, Artificial Sequence
  clone 8 light chain
QSVLTQPPSVSGAPGQRVTISCTGSSSDIGAGYDVHWYQQLPGTAPKLLIFANTNRPSGVPDRFSGSKSGASASLAITGLQADDEADYYCQSYDRSLSHVFGTGTKVTVLG

SEQ ID NO: 21 - protein, 123 aa, Artificial Sequence
  clone 9 heavy chain
QVTLKESGGGVVQSGRSLRLSCAASGFTFSSYTMHWVRQAPGKGLEWVSSITGGSSYVDYSASVKGRFTISRDNAQSSLYLQMNSLRAEDTAVYYCARDDYGSGSYSNWFDPWGQGTLVTVSS

SEQ ID NO: 22 - protein, 111 aa, Artificial Sequence
  clone 9 light chain
QSVLTQPPSVSGAPGQRVTISCTGSSSNIGAGYDVHWYQQLPGRAPKLLIYANTNRPSGVADRFSGSKSGASASLAITGLQADDEADYYCQSYDRSLSHVFGTGTKVTVLG

SEQ ID NO: 23 - protein, 125 aa, Artificial Sequence
  clone 13 heavy chain
EVQLVESGGGLVKPGGSLRLSCAASGFTFTSYRMHWVRQAPGKGLEWVSSITGGGNYIEYADSVKGRFTISRDNAKNSLDLQMNSLRAEDTAIYYCARDMYGLGSYYSPNYFDSWGQGTLVTVSS

SEQ ID NO: 24 - protein, 111 aa, Artificial Sequence
  clone 13 light chain
QSVLTQPPSVSGAPGQRVTISCTGSSSNIGAGYDVHWYQQLPGRAPKLLIFANTNRPSGVPDRFSGSKSGASASLAITGLQADDEADYYCQSYDRSLSHVFGTGTKVTVLG

SEQ ID NO: 25 - protein, 123 aa, Artificial Sequence
  clone 16 heavy chain
EVQLVESGGGLVKPGGSLRLSCAGSGFTFSSYTMHWVRQAPGKGLEWVSSITGGSSYVDYSASVKGRFTISRDNAQSSLYLQMNSLRAEDTAVYYCARDDYGSGSYSNWFDPWGRGTTVTVSS

SEQ ID NO: 26 - protein, 111 aa, Artificial Sequence
  clone 16 light chain
QPVLTQPLSASGTPGQRVTISCTGSSSNIGAGYDVHWYQQLPGRAPKLLIFANTNRPSGVPDRFSGSKSGTSASLAITGLQAEDEADYYCQSYDRSLSHVFGTGTKVTVLG

SEQ ID NO: 27 - protein, 123 aa, Artificial Sequence
  clone 33 heavy chain
QVTLKESGGGLVKPGGSLRLSCAASGFRLSSYGMNWVRQAPGKGLEWVSSISASSSFINYADSVRDRFTISRDNAKNSLYLQMNSLRAEDTAVYYCARDDYGSGSYSNWFDPWGQGTLVTVSS

SEQ ID NO: 28 - protein, 111 aa, Artificial Sequence
  clone 33 light chain
QSVLTQPPSVSGAPGQRVTISCTGNSSNLGAGYDVHWYQQLPGRAPKLLIFANTNRPSGVPDRFSGSKSGASASLAITSLQADDEADYYCQSYDRSLSHVFGTGTKVTVLG

SEQ ID NO: 29 - protein, 123 aa, Artificial Sequence
  clone 6m heavy chain
EVQLVESGGGLVKPGGSLRLSCAGSGFTFSSYTMHWVRQAPGKGLEWVSSITGGSSYVDYSASVKGRFTISRDNAQSSLYLQMNSLRAEDTAVYYCARDDYGSGSYSNWFDPWGQGTLVTVSS

SEQ ID NO: 30 - protein, 111 aa, Artificial Sequence
  clone 6m light chain
QSVLTQPPSASGTPGQRVTISCTGSSSNIGAGYDVHWYQQLPGAAPRLLMFGNSNRPSGVPDRFSGSKSGTSASLAITGLQADDEADYYCQSYDRSLSHVFGTGTKVTVLG

SEQ ID NO: 31 - protein, 123 aa, Artificial Sequence
  clone 11m heavy chain
EVQLVESGGGLVKPGGSLRLSCAASGFTFTSYRMHWVRQAPGKGLEWVSSITGGGNYIEYADSVKGRFTISRDNAQSSLYLQMNSLRAEDTAVYYCARDDYGSGSYSNWFDPWGQGTLVTVSS

SEQ ID NO: 32 - protein, 123 aa, Artificial Sequence
  clone 12m heavy chain
EVQLVESGGGLVKPGGSLRLSCAGSGFAFSSYTMHWVRQAPGKGLEWVSSITGGSSYLDYAHSVKGRFTISRDNGQNSLFLQMNSLRTEDTAVYYCARDDYGSGSYSNYFDPWGQGTLVTVSS

SEQ ID NO: 33 - protein, 111 aa, Artificial Sequence
  clone 12m light chain
QSVLTQPPSVSGAPGQRVTISCTGSSSNIGAGYDVHWYQQVPGTAPKLLIFGSTNRPSGVPDRFSGSKSGASASLAITGLQTEDEADYYCQSYDRSLSHVFGTGTKVTVLG

SEQ ID NO: 34 - DNA, 369 bp, Artificial Sequence
  clone 8 heavy chain
gaggtgcagctggtggagtctgggggaggcctgatacagcctggggggtccctgagactctcctgtgcaggctctggattcaccttcagtagctataccatgcactgggtccgccaggctccagggaaggggctggagtgggtctcgtccataactggtggcagtagttatgtcgactactcagcctcagtgaagggccgattcaccatctccagagacaacgcccagagctcactttatctgcaaatgaacagcctgagagccgaggacacggccgtgtattactgtgcgagagatgattatggttcggggagttattccaactggttcgacccctggggccagggaaccctggtcaccgtctcctca

SEQ ID NO: 35 - DNA, 333 bp, Artificial Sequence
  clone 8 light chain
cagtctgtcctgacgcagccgccctcagtgtctggggccccagggcagagggtcaccatctcctgcactgggagcagctccgacatcggggcaggttatgatgtacactggtaccagcaacttccaggaacagcccccaaactcctcatctttgctaacaccaatcggccctcaggggtccctgatcgattctctggctccaagtctggcgcctctgcctccctggccatcactggcctccaggctgacgatgaggctgattattactgccagtcctatgaccgcagcctgagtcatgtcttcggaactgggaccaaggtcaccgtcctaggc

SEQ ID NO: 36 - DNA, 369 bp, Artificial Sequence
  clone 9 heavy chain
caggtcaccttgaaggagtctgggggaggcgtggtccagtctgggaggtccctgagactctcctgtgcagcctctggattcaccttcagtagctataccatgcactgggtccgccaggctccagggaaggggctggagtgggtctcgtccataactggtggcagtagttatgtcgactactcagcctcagtgaagggccgattcaccatctccagagacaacgcccagagctcactttatctgcaaatgaacagcctgagagccgaggacacggctgtgtattactgtgcgagagatgattatggttcggggagttattccaactggttcgacccctggggccagggaaccctggtcaccgtctcctca

SEQ ID NO: 37 - DNA, 333 bp, Artificial Sequence
  clone 9 light chain
cagtctgtgctgacgcagccgccctcagtgtctggggccccagggcagagggtcaccatctcctgcactgggagcagctccaacatcggggcaggttatgatgtacactggtaccagcagcttccaggaagagcccccaaactcctcatctatgctaacaccaatcggccctcaggggtcgctgaccgattctctggctccaagtctggcgcctctgcctccctggccatcactggcctccaggctgacgatgaggctgattattactgccagtcctatgaccgcagcctgagtcatgtcttcggaactgggaccaaggtcaccgtcctaggc

SEQ ID NO: 38 - DNA, 375 bp, Artificial Sequence
  clone 13 heavy chain
gaggtgcagctggtggagtctgggggaggcctggtcaagcctggggggtccctgagactctcctgtgcagcctctggattcaccttcactagttataggatgcattgggtccgccaggctccagggaaggggctggagtgggtctcatcaattactggtggtggtaattatatagagtacgcagactcagtgaagggccggttcaccatctccagagacaacgccaagaactcactggatctgcaaatgaacagcctgagagccgaggacacggctatttattactgtgcgagagatatgtatggtttggggagttattattcgcctaactacttcgactcctggggccagggaaccctggtcaccgtctcctca

SEQ ID NO: 39 - DNA, 333 bp, Artificial Sequence
  clone 13 light chain
cagtctgtgctgacgcagccgccctcagtgtctggggccccagggcagagggtcaccatctcctgcactgggagcagctccaacatcggggcaggttatgatgtacactggtaccagcagcttccaggaagagcccccaaactcctcatctttgctaacaccaatcggccctcaggggtccctgaccgattctctggctccaagtctggcgcctctgcctccctggccatcactggcctccaggctgacgatgaggctgattattactgccagtcctatgaccgcagcctgagtcatgtcttcggaactgggaccaaggtcaccgtcctaggc

SEQ ID NO: 40 - DNA, 369 bp, Artificial Sequence
  clone 16 heavy chain
gaggtgcagctggtggagtctgggggaggcctggtcaagcctggggggtccctgagactctcctgtgcaggctctggattcaccttcagtagctataccatgcactgggtccgccaggctccagggaaggggctggagtgggtctcgtccataactggtggcagtagttatgtcgactactcagcctcagtgaagggccgattcaccatctccagagataacgcccagagctcactttatctgcaaatgaacagcctgagagccgaggacacggctgtgtattactgtgcgagagatgattatggttcggggagttattccaactggttcgacccctggggccggggaaccacggtcaccgtctcctca

SEQ ID NO: 41 - DNA, 333 bp, Artificial Sequence
  clone 16 light chain
cagcctgtgctgactcagccactctcagcgtctgggacccccgggcagagggtcaccatctcctgcactgggagcagctccaacatcggggcaggttatgatgtacactggtaccagcagcttccaggaagagcccccaaactcctcatctttgctaacaccaatcggccctcaggggtccctgaccgattctctggctccaagtcgggcacctcagcctccctggccatcactgggctccaggctgaggatgaggctgattattactgccagtcctatgaccgcagcctgagtcatgtcttcggaactgggaccaaggtcaccgtcctaggc

SEQ ID NO: 42 - DNA, 369 bp, Artificial Sequence
  clone 33 heavy chain
caggtcaccttgaaggagtctgggggcggcctggttaagcctggggggtccctgagactctcgtgtgcagcctctgggttcaggctcagtagctatggcatgaactgggtccgccaggctccagggaaggggctggagtgggtctcatccatttctgctagtagtagttttataaactatgcagactcagtgagggaccgattcaccatctccagagacaacgccaagaactcactgtatctgcaaatgaacagcctgagagccgaggacacggctgtgtattactgtgcgagagatgattatggttcggggagttattccaactggttcgacccctggggccagggaaccctggtcaccgtctcctca

SEQ ID NO: 43 - DNA, 333 bp, Artificial Sequence
  clone 33 light chain
cagtctgtgctgacgcagccgccctcagtgtctggggccccagggcagagggtcaccatttcctgcactgggaacagctccaacctcggggcaggttatgatgtacactggtaccagcagcttccaggaagagcccccaaactcctcatctttgctaacaccaatcggccctcaggggtccctgaccgattctctggctccaagtctggcgcctctgcctccctggccatcactagcctccaggctgacgatgaggctgattattactgccagtcctatgaccgcagcctgagtcatgtcttcggaactgggaccaaggtcaccgtcctaggc

SEQ ID NO: 44 - DNA, 369 bp, Artificial Sequence
  clone 6m heavy chain
gaggtgcagctggtggagtctgggggaggcctggtcaagcctggggggtccctgagactctcctgtgcaggctctggattcaccttcagtagctataccatgcactgggtccgccaggctccagggaaggggctggagtgggtctcgtccataactggtggcagtagttatgtcgactactcagcctcagtgaagggccgattcaccatctccagagacaacgcccagagctcactttatctgcaaatgaacagcctgagagccgaggacacggctgtatattactgtgcgagagatgattatggttcggggagttattccaactggttcgacccctggggccagggaaccctggtcaccgtctcctca

SEQ ID NO: 45 - DNA, 333 bp, Artificial Sequence
  clone 6m light chain
cagtctgtgctgacgcagccgccctcagcgtctgggacccccgggcagagggtcaccatctcctgcactgggagcagctccaacatcggggcaggttatgatgtacactggtatcagcagcttccgggagcagcccccagactcctcatgtttggtaacagcaatcggccctcgggggtacctgaccgcttctctggctccaagtctggcacctccgcctccctggccatcactggcctccaggctgacgatgaggctgattattactgccagtcctatgaccgcagcctgagtcatgtcttcggaactgggaccaaggtcaccgtcctaggc

SEQ ID NO: 46 - DNA, 369 bp, Artificial Sequence
  clone 11m heavy chain
gaggtgcagctggtggagtctgggggaggcctggtcaagcctggggggtccctgagactctcctgtgcagcctctggattcaccttcactagttataggatgcattgggtccgccaggctccagggaaggggctggagtgggtctcatcaattactggtggtggtaattatatagagtacgcagactcagtgaagggccgattcaccatctccagagacaacgcccagagctcactttatctgcaaatgaacagcctgagagccgaggacacggctgtgtattactgtgcgagagatgattatggttcggggagttattccaactggttcgacccctggggccagggaaccctggtcaccgtctcctca

SEQ ID NO: 47 - DNA, 369 bp, Artificial Sequence
  clone 12m heavy chain
gaggtgcagctggtggagtctgggggaggcctggtcaagcctggggggtccctgagactttcctgtgctggctctggattcgccttcagtagttacactatgcactgggtgcgccaggctccagggaaggggctggagtgggtctcatccatcactggcggcagtagttacctagactacgcacactcagtgaagggccgattcaccatctccagagacaatggccagaactcactgtttctgcaaatgaacagcctgaggaccgaggacacggctgtatattactgtgcgagagatgactatggttcggggagttattccaactacttcgacccctggggccagggaaccctggtcaccgtctcctca

SEQ ID NO: 48 - DNA, 333 bp, Artificial Sequence
  clone 12m light chain
cagtctgtgctgacgcagccgccctcagtgtctggggccccagggcagagggtcaccatctcctgcactgggagcagctccaacatcggggcaggttatgatgtacactggtaccagcaggttccaggaacggcccccaaactcctcatctttggtagcaccaatcggccctcaggggtccctgaccgattctctggctccaagtctggcgcctcagcctccctggccatcactgggctccagactgaggatgaggctgattattactgccagtcctatgaccgcagcctgagtcatgtcttcggaactgggaccaaggtcaccgtcctaggc

SEQ ID NO: 49 - DNA, 369 bp, Artificial Sequence
  clone 1 heavy chain
gaggtgcagctggtggagtctgggggaggcctggtcaagcctggggggtccctgagactctcctgtgcagcctctggattcacgttcagtagctataccatgcactgggtccgccaggctccagggaaggggctggagtgggtctcgtccataactggtggcagtagttatgtcgactactcagcctcagtgaagggccgattcaccatctccagagacaacgctcagagctcactttatctgcaaatgaacagcctgagagccgaggacacggctgtgtattactgtgcgagagatgattatggttcggggagttattccaactggttcgacccctggggccagggaaccctggtcaccgtctcctca

SEQ ID NO: 50 - DNA, 333 bp, Artificial Sequence
  clone 1 light chain
cagtctgtgctgacgcagccgccctcagtgtctggggccccagggcagagggtcaccatctcctgcactgggagcagctccaacatcggggcaggttatgatgtacactggtaccagcaggttccaggaacagcccccaaactcctcatctttggtagcaccaatcggccctcaggggtccctgaccgattctctggctccaagtctggcacctcagcctccctggccatcactggcctccaggctgacgatgaggctgattattactgccagtcctatgaccgcagcctgagtcatgtcttcggaactgggaccaaggtcaccgtcctaggc

SEQ ID NO: 51 - DNA, 369 bp, Artificial Sequence
  clone 2 heavy chain
gaggtgcagctggtggagtctgggggaggcgtggtccagtctgggaggtccctgagactctcctgtgcaggctctggattcaccttcagtagctataccatgcactgggtccgccaggctccagggaaggggctggagtgggtctcgtccataactggtggcagtagttatgtcgactactcagcctcagtgaagggccgattcaccatctccagagacaacgcccagagctcactttatctgcaaatgaacagcctgagagccgaggacacggctgtgtattactgtgcgagagatgattatggttcggggagttattccaactggttcgacccctggggccagggaaccctggtcaccgtctcctca

SEQ ID NO: 52 - DNA, 333 bp, Artificial Sequence
  clone 2 light chain
cagtctgtcctgacgcagccgccctcagtgtctggggccccagggcagagggtcaccatctcctgcactgggagcagctccaacatcggggcaggttatgatgtacactggtaccagcaggttccaggaacagcccccaaactcctcatctttggtagcaccaatcggccctcaggggtccctgaccgattctctggctccaagtctggcgcctcagcctccctggccatcactgggctccagactgaggatgaggctgattattactgccagtcctatgaccgcagcctgagtcatgtcttcggaactgggaccaaggtcaccgtcctaggc

SEQ ID NO: 53 - DNA, 369 bp, Artificial Sequence
  clone 3 heavy chain
gaggtgcagctggtggagtctgggggaggcctggtcaagcctggggggtccctgagactctcctgtgcaggctctggattcaccttcagtagctataccatgcactgggtccgccaggctccagggaaggggctggagtgggtctcgtccataactggtggcagtagttatgtcgactactcagcctcagtgaagggccgattcaccatctccagagacaacgcccagagctcactttatctgcaaatgaacagcctgagagccgaggacacggctgtgtattactgtgcgagagatgattatggttcggggagttattccaactggttcgacccctggggccagggaaccctggtcaccgtctcctca

SEQ ID NO: 54 - DNA, 333 bp, Artificial Sequence
  clone 3 light chain
cagtctgtgctgacgcagccgccctcagtgtctggggccccagggcagagggtcaccatctcctgcactgggagcagctccaacatcggggcaggttacgatgtacactggtaccagcaggttccaggaacagcccccaaactcctcatctttggtagcaccaatcggccctcaggggtccctgaccgattctctggttccaagtctggcgcctctgcctccctggccatcactggcctccaggctgacgatgaggctgattattactgccagccctatgaccgcagcctgagtcatgtcttcggaactgggaccaaggtcaccgtcctacgc

SEQ ID NO: 55 - DNA, 369 bp, Artificial Sequence; identical to SEQ ID NO: 53
  clone 4 heavy chain

SEQ ID NO: 56 - DNA, 333 bp, Artificial Sequence
  clone 4 light chain
cagtctgtgctgacgcagccgccctcagtgtctggggccccagggcagagggtcaccatctcctgcactgggagcagctccaacatcggggcaggttacgatgtacactggtaccagcaggttccaggaacagcccccaaactcctcatctttggtagcaccaatcggccctcaggggtccctgaccgattctctggctccaagtctggcgcctctgcctccctggccatcactggcctccaggctgacgatgaggctgattattactgccagtcctatgaccgcagcctgagtcatgtcttcggaactgggaccaaggtcaccgtcctaggc

SEQ ID NO: 57 - DNA, 369 bp, Artificial Sequence; identical to SEQ ID NO: 53
  clone 5 heavy chain

SEQ ID NO: 58 - DNA, 333 bp, Artificial Sequence
  clone 5 light chain
cagtctgtgctgacgcagccgccctcagtgtctggggccccagggcagagggtcaccatctcctgcactgggagcagctccaacatcggggcaggttatgatgtacactggtatcagcagcttccgggagcagcccccagactcctcatgtttggtaacagcaatcggccctcgggggtacctgaccgcttctctggctccaagtctggcacctccgcctccctggccatcactggtctccaggctgaggatgaggctgattattactgccagtcctatgaccgcagcctgagtcatgtcttcggaactggcaccaaggtgaccgtcctcggc

SEQ ID NO: 59 - DNA, 333 bp, Artificial Sequence
  clone 6 light chain
tcctatgagctgactcagccaccctcagcgtctgggacccccgggcagagggtcaccatctcctgcactgggagcagctccaacatcggggcaggttatgatgtacactggtatcagcagcttccgggagcagcccccagactcctcatgtttggtaacagcaatcggccctcgggggtacctgaccgcttctctggctccaagtctggcacctccgcctccctggccatcactggcctccaggctgacgatgaggctgattattactgccagtcctatgaccgcagcctgagtcatgtcttcggaactgggaccaaggtcaccgtcctaggc

SEQ ID NO: 60 - DNA, 369 bp, Artificial Sequence
  clone 7 heavy chain
caggtgcagctggtgcagtctgggggaggcttgatacagcctggggggtccctgagactctcctgtgcaggctctggattcaccttcagtagctataccatgcactgggtccgccaggctccagggaaggggctggagtgggtctcgtccataactggtggcagtagttatgtcgactactcagcctcagtgaagggccgattcaccatctccagagacaacgcccagagctcactttatctgcaaatgaacagcctgagagccgaggacacggccgtgtattactgtgcgagagatgattatggttcggggagttattccaactggttcgacccctggggccagggaaccctggtcaccgtctcctca

SEQ ID NO: 61 - DNA, 333 bp, Artificial Sequence
  clone 7 light chain
cagtctgtgctgacgcagccgccctcagtgtctggggccccagggcagagggtcaccatctcctgcactgggagcagctccaacatcggggcaggttatgatgtacactggtaccagcaacttccaggaacagcccccaaactcctcatctttgctaacaccaatcggccctcaggggtccctgatcgattctctggctccaagtctggcgcctctgcctccctggccatcactggcctccaggctgacgatgaggctgattattactgccagtcctatgaccgcagcctgagtcatgtcttcggaactgggaccaaggtcaccgtcctaggc

SEQ ID NO: 62 - DNA, 426 bp, Artificial Sequence
  clone 9m heavy chain
tgctgtgggtgagtggtacctgtggggaggtgcagctggtggagtctgggggaggcgtggtccagtctgggaggtccctgagactctcctgtgcagcctctggattcaccttcagtagctataccatgcactgggtccgccaggctccagggaaggggctggagtgggtctcgtccataactggtggcagtagttatgtcgactactcagcctcagtgaagggccgattcaccatctccagagacaacgcccagagctcactttatctgcaaatgaacagcctgagagccgaggacacggctgtgtattactgtgcgagagatgattatggttcggggagttattccaactggttcgacccctggggccagggaaccctggtcaccgtctcctcagcctccaccaagggcccatcggtcttccccc

SEQ ID NO: 63 - DNA, 369 bp, Artificial Sequence
  clone 10 heavy chain
gaggtgcagctggtggagtctgggggaggcctggtcaagcctggggggtccctgagactctcctgtgcaggctctggattcaccttcagtagctataccatgcactgggtccgccaggctccagggaaggggctggagtgggtctcgtccataactggtggcagtagttatgtcgactactcagcctcagtgaagggccgattcaccatctccagagacaacgcccagagctcactttatctgcaaatgaacagcctgagagccgaggacacggctgtgtattactgtgcgagagatgattatggttcggggagttattctaactggttcgacccctggggccagggaaccctggtcaccgtctcctca

SEQ ID NO: 64 - DNA, 333 bp, Artificial Sequence
  clone 10 light chain
cagtctgtgctgacgcagccgccctcagtgtctggggccccagggcagagggtcaccatttcctgcactgggaacagctccaacctcggggcaggttatgatgtacactggtaccagcaacttccaggaacagcccccaaactcctcatctatgctaacaccaatcggccctcaggggtccctgaccgattctctggctccaagtctggcgcctcagcctccctggccatcactgggctccagactgaggatgaggctgattattactgccagtcctatgaccgcagcctgagtcatgtcttcggaactgggaccaaggtcaccgtcctaggc

SEQ ID NO: 65 - DNA, 333 bp, Artificial Sequence
  clone 11 light chain
cagactgtggtgactcaggagccctcagtgtctggggccccagggcagagggtcaccatctcctgcactgggagcagctccaacatcggggcaggttatgatgtacactggtaccagcagcttccaggaagagcccccaaactcctcatctttgctaacaccaatcggccctcaggggtccctgaccgattctctggctccaagtctggcgcctctgcctccctggccatcactggcctccaggctgacgatgaggctgattattactgccagtcctatgaccgcagcctgagtcatgtcttcggaactgggaccaaggtcaccgtcctaggc

SEQ ID NO: 66 - DNA, 333 bp, Artificial Sequence
  clone 12 light chain
cagcctgtgctgactcagccaccctcagtgtctggggccccagggcagagggtcaccatctcctgcactgggagcagctccaacatcggggcaggttatgatgtacactggtaccagcaggttccaggaacggcccccaaactcctcatctttggtagcaccaatcggccctcaggggtccctgaccgattctctggctccaagtctggcgcctcagcctccctggccatcactgggctccagactgaggatgaggctgattattactgccagtcctatgaccgcagcctgagtcatgtcttcggaactgggaccaaggtcaccgtcctaggc

SEQ ID NO: 67 - DNA, 369 bp, Artificial Sequence
  clone 14 heavy chain
caggtcaccttgaaggagtctgggggaggcctggtcaagcctggggggtccctgagactctcctgtgcaggctctggattcaccttcagtagctataccatgcactgggtccgccaggctccagggaaggggctggagtgggtctcgtccataactggtggcagtagttatgtcgactactcagcctcagtgaagggccgattcaccatctccagagacaacgccaagaactcactgtttctgcaaatgaacagcctgagagccgaggacacggctgtgtattactgtgcgagagatgattatggttcggggagttattccaactggttcgacccctggggccagggaaccctggtcaccgtctcctca

SEQ ID NO: 68 - DNA, 368 bp, Artificial Sequence
  clone 14m heavy chain
aggtgcagctggtggagtctgggggaggcctggtcaagcctggggggtccctgagactctcctgtgcaggctctggattcaccttcagtagctataccatgcactgggtccgccaggctccagggaaggggctggagtgggtctcgtccataactggtggcagtagttatgtcgactactcagcctcagtgaagggccgattcaccatctccagagacaacgccaagaactcactgtttctgcaaatgaacagcctgagagccgaggacacggctgtgtattactgtgcgagagatgattatggttcggggagttattccaactggttcgacccctggggccagggaaccctggtcaccgtctcctca

SEQ ID NO: 69 - DNA, 333 bp, Artificial Sequence
  clone 14 light chain
cagtctgtgctgacgcagccgccctcagtttctggggccccagggcagagggtcaccatctcctgcactgggagcagctccaacatcggggcaggttatgatgtacactggtaccagcagcttccaggaagagcccccaaactcctcatctttgctaacaccaatcggccctcaggggtccctgaccgattctctggctccaagtctggcgcctctgcctccctggccatcactggcctccaggctgacgatgaggctgattattactgccagtcctatgaccgcagcctgagtcatgtcttcggaactgggaccaaggtcaccgtcctaggc

SEQ ID NO: 70 - DNA, 375 bp, Artificial Sequence
  clone 15 heavy chain
gaggtgcagctggtggagtctgggggaggcgtggtccagcctgggaggtccctgagactcgcctgtgcagcctctggattcaccttcaatagctatgctatgcactgggtccgccaggctccagggaaggggctggagtgggtctcgtccataactggtggcagtagttatgtcgactactcagcctcagtgaagggccgattcaccatctccagagacaacgcccagagctcactttatctgcaaatgaacagcctgagagccgaggacacggctgtgtattactgtgcgagagatatgtatggtttggggagttattattcgcctaactacttcgacccctggggccagggaaccctggtcactgtctcctca

SEQ ID NO: 71 - DNA, 333 bp, Artificial Sequence
  clone 15 light chain
tcctatgagctgactcagccaccctcagtgtctggggccccagggcagagggtcaccatctcctgcactgggagcagctccaacatcggggcaggttatgatgtacactggtaccagcagcttccaggaagagcccccaaactcctcatctttgctaacaccaatcggccctcaggggtccctgaccgattctctggctccaagtctggcacctccgcctccctggccatcactggtctccaggctgaggatgaggctgattattactgccagtcctatgacagtagcctgagttatgtcttcggaactgggaccaaggtcaccgtcctaggc

SEQ ID NO: 72 - DNA, 333 bp, Artificial Sequence
  clone 15m light chain
cagtctgtgctgacgcagccgccctcagtgtctggggccccagggcagagggtcaccatctcctgcactgggagcagctccaacatcggggcaggttatgatgtacactggtaccagcagcttccaggaagagcccccaaactcctcatctttgctaacaccaatcggccctcaggggtccctgaccgattctctggctccaagtctggcacctccgcctccctggccatcactggtctccaggctgaggatgaggctgattattactgccagtcctatgacagtagcctgagttatgtcttcggaactgggaccaaggtcaccgtcctaggc

SEQ ID NO: 73 - DNA, 333 bp, Artificial Sequence
  clone 16m light chain
cagtctgtgctgacgcagccgctctcagcgtctgggacccccgggcagagggtcaccatctcctgcactgggagcagctccaacatcggggcaggttatgatgtacactggtaccagcagcttccaggaagagcccccaaactcctcatctttgctaacaccaatcggccctcaggggtccctgaccgattctctggctccaagtcgggcacctcagcctccctggccatcactgggctccaggctgaggatgaggctgattattactgccagtcctatgaccgcagcctgagtcatgtcttcggaactgggaccaaggtcaccgtcctaggc

SEQ ID NO: 74 - DNA, 369 bp, Artificial Sequence
  clone 17 heavy chain
gaggtgcagctggtggagtctgggggaggcttggtacagcctggagggtccctgagactcgcctgtgcagcctctggattcaccttcagtagctataccatgcactgggtccgccaggctccagggaaggggctggagtgggtctcgtccataactggtggcagtagttatgtcgactactcagcctcagtgaagggccgattcaccatctccagagacaacgcccagagctcactttatctgcaaatgaacagcctaagagccgaggacacggctgtgtattactgtgcgagagatgattatggttcggggagttattccaactggttcgacccctggggccagggaaccctggtcaccgtctcctca

SEQ ID NO: 75 - DNA, 333 bp, Artificial Sequence
  clone 17 light chain
tcctatgagctgactcagccaccctcagtgtctggggccccagggcagagggtcaccatctcctgcactgggagcagctccaacatcggggcaggttatgatgtacactggtaccagcagcttccaggaagagcccccaaactcctcatctttgctaacaccaatcggccctcaggggtccctgaccgattctctggctccaagtctggcgcctctgcctccctggccatcactggcctccaggctgaggatgaggctgattattactgccagtcctatgaccgcagcctgagtcatgtcttcggaactgggaccaaggtcaccgtcctaggc

SEQ ID NO: 76 - DNA, 333 bp, Artificial Sequence
  clone 17m light chain
cagtctgtgctgacgcagccgccctcagtgtctggggccccagggcagagggtcaccatctcctgcactgggagcagctccaacatcggggcaggttatgatgtacactggtaccagcagcttccaggaagagcccccaaactcctcatctttgctaacaccaatcggccctcaggggtccctgaccgattctctggctccaagtctggcgcctctgcctccctggccatcactggcctccaggctgaggatgaggctgattattactgccagtcctatgaccgcagcctgagtcatgtcttcggaactgggaccaaggtcaccgtcctaggc

SEQ ID NO: 77 - DNA, 375 bp, Artificial Sequence
  clone 18 heavy chain
caggtcaccttgaaggagtctgggggaggcctggtcaagcctggggggtccctgagactctcctgtgcagcctctggattcaccttcactagttataggatgcattgggtccgccaggctccagggaaggggctggagtgggtctcatcaattactggtggtggtaattatatagagtacgcagactcagtgaagggccggttcaccatctccagagacaacgccaagaactcactggatctgcaaatgaacagcctgagagccgaggacacggctatttattactgtgcgagagatatgtatggtttggggagttattattcgcctaactacttcgacccctggggccagggaaccctggtcaccgtctcctca

SEQ ID NO: 78 - DNA, 375 bp, Artificial Sequence
  clone 18m heavy chain
gaggtgcagctggtggagtctgggggaggcctggtcaagcctggggggtccctgagactctcctgtgcagcctctggattcaccttcactagttataggatgcattgggtccgccaggctccagggaaggggctggagtgggtctcatcaattactggtggtggtaattatatagagtacgcagactcagtgaagggccggttcaccatctccagagacaacgccaagaactcactggatctgcaaatgaacagcctgagagccgaggacacggctatttattactgtgcgagagatatgtatggtttggggagttattattcgcctaactacttcgacccctggggccagggaaccctggtcaccgtctcctca

SEQ ID NO: 79 - DNA, 333 bp, Artificial Sequence
  clone 18 light chain
tcctatgagctgactcagccactctcagtgtctggggccccagggcagagggtcaccatttcctgcactgggagcagctccaacatcggggcaggttatgatgtacactggtaccagcaggttccaggaacagcccccaaactcctcatctttggtagcaccaatcggccctcaggggtccctgaccgattctctggctccaagtctggcgcctctgcctccctggccatcactggcctccaggctgacgatgaggctgattattactgccagtcctatgaccgcagcctgagtcatgtcttcggaactgggaccaaggtcaccgtcctaggc

SEQ ID NO: 80 - DNA, 333 bp, Artificial Sequence
  clone 18m light chain
cagtctgtgctgacgcagccgctctcagtgtctggggccccagggcagagggtcaccatttcctgcactgggagcagctccaacatcggggcaggttatgatgtacactggtaccagcaggttccaggaacagcccccaaactcctcatctttggtagcaccaatcggccctcaggggtccctgaccgattctctggctccaagtctggcgcctctgcctccctggccatcactggcctccaggctgacgatgaggctgattattactgccagtcctatgaccgcagcctgagtcatgtcttcggaactgggaccaaggtcaccgtcctaggc

SEQ ID NO: 81 - DNA, 375 bp, Artificial Sequence
  clone 19 heavy chain
gaggtgcagctggtggagtctgggggaggcctggtcaagcctggggggtccctgagactctcctgtgcagcctctggattcaccttcactagttataggatgcattgggtccgccaggctccagggaagaggctggagtgggtctcatcaattactggtggtggtaattatatagagtacgcagactcagtgaagggccggttcaccatctccagagacaacgccaagaactcactggatctgcaaatgaacagcctgagagccgaggacacggctatttattactgtgcgagagatatgtatggtttggggagttattattcgcctaactacttcgacccctggggccagggaaccctggtcaccgtctcctca

SEQ ID NO: 82 - DNA, 333 bp, Artificial Sequence
  clone 19 light chain
cagtctgtgctgacgcagccgccctcagtgtctggggctccagggcagagggtcaccatctcctgcactgggagcagctccaacatcggggcaggttatgatgtacactggtaccagcaggttccaggaacagcccccaaactcctcatctttggtagcaccaatcggccctcaggggtccctgaccgattctctggctccaagtctggcgcctcagcctccctggccatcactgggctccagactgaggatgaggctgattattactgccagtcctatgaccgcagcctgagtcatgtcttcggaactgggaccaaggtcaccgtcctaggc

SEQ ID NO: 83 - DNA, 375 bp, Artificial Sequence; identical to SEQ ID NO: 78
  clone 20 heavy chain

SEQ ID NO: 84 - DNA, 333 bp, Artificial Sequence
  clone 20 light chain
cagcctgtgctgactcagccaccctcagtgtctggggccccagggcagagggtcaccatctcctgcactgggagcagctccaacatcggggcaggttatgatgtacactggtaccagcaggttccaggaacagcccccaaactcctcatctttggtagcaccaatcggccctcaggggtccctgaccgattctctggctccaagtctggcgcctcagcctccctggccatcactgggctccagactgaggatgaggctgattattactgccagtcctatgaccgcagcctgagtcatgtcttcggaactgggaccaaggtcaccgtcctaggc

SEQ ID NO: 85 - DNA, 333 bp, Artificial Sequence
  clone 20m light chain
cagtctgtgctgacgcagccgccctcagtgtctggggccccagggcagagggtcaccatctcctgcactgggagcagctccaacatcggggcaggttatgatgtacactggtaccagcaggttccaggaacagcccccaaactcctcatctttggtagcaccaatcggccctcaggggtccctgaccgattctctggctccaagtctggcgcctcagcctccctggccatcactgggctccagactgaggatgaggctgattattactgccagtcctatgaccgcagcctgagtcatgtcttcggaactgggaccaaggtcaccgtcctaggc

SEQ ID NO: 86 - DNA, 375 bp, Artificial Sequence; identical to SEQ ID NO: 77
  clone 21 heavy chain

SEQ ID NO: 87 - DNA, 375 bp, Artificial Sequence; identical to SEQ ID NO: 78
  clone 21m heavy chain

SEQ ID NO: 88 - DNA, 375 bp, Artificial Sequence; identical to SEQ ID NO: 78
  clone 21 light chain

SEQ ID NO: 89 - DNA, 375 bp, Artificial Sequence
  clone 22 heavy chain
gaggtgcagctggtggagtctgggggaggcctggtcaagcctggggggtccctgagactctcctgtgcagcctctggattcaccttcactagttataggatgcattgggtccgccaggctccagggaaggggctggagtgggtctcatcaattactggtggtggtaattatatagagtacgcagactcagtgaagggccggttcaccatctccagagacaacgccaagaactcactggacctgcaaatgaacagcctgagagccgaggacacggctatttattactgtgcgagagatatgtatggtttggggagttattattcgcctaactacttcgacccctggggccagggaaccctggtcactgtctcctca

SEQ ID NO: 90 - DNA, 333 bp, Artificial Sequence; identical to SEQ ID NO: 69
  clone 22 light chain

SEQ ID NO: 91 - DNA, 375 bp, Artificial Sequence
  clone 23 heavy chain
caggtccagctggtacagtctgggggaggcctggtcaagcctggggggtccctgagactctcctgtgcagcctctggattcaccttcactagttataggatgcattgggtccgccaggctccagggaaggggctggagtgggtctcatcaattactggtggtggtaattatatagagtacgcagactcagtgaagggccggttcaccatctccagagacaacgccaagaactcactggatctgcaaatgaacagcctgagagccgaggacacggctatttattactgtgcgagagatatgtatggtttggggagttattattcgcctaactacttcgacccctggggccagggaaccacggtcaccgtctcctca

SEQ ID NO: 92 - DNA, 333 bp, Artificial Sequence
  clone 23 light chain
cagtctgtgttgacgcagccgccctcagtgtctggggccccagggcagagggtcaccatctcctgcactgggagcagctccaacatcggggcaggttatgatgtacactggtaccagcagcttccaggaagagcccccaaactcctcatctttgctaacaccaatcggccctcaggggtccctgaccgattctctggctccaagtctggcgcctctgcctccctggccatctctgggctccaggctgaggatgaggctcattattactgccagtcctatgacaggagcctgaatgtggttttcggcggagggaccgagctgaccgtcctaggc

SEQ ID NO: 93 - DNA, 375 bp, Artificial Sequence; identical to SEQ ID NO: 78
  clone 24 heavy chain

SEQ ID NO: 94 - DNA, 336 bp, Artificial Sequence
  clone 24 light chain
cagtctgtgctgacgcagccgccctcagtgtctggggccccagggcagagggtcaccatctcctgcactgggagcagctccaacatcggggcaggttatgatgtacactggtaccagcaggttccaggaacagcccccaaactcctcatctttggtagcaccaatcggccctcaggggtccctgaccgattctctggctccaagtctggcgcctcagcctccctggccatcactgggctccagactgaggatgaggctgattattattgccagtcctatgacagaagcctgagtgcttgggtgttcggcggagggaccaagctgaccgtcctaggc

SEQ ID NO: 95 - DNA, 375 bp, Artificial Sequence; identical to SEQ ID NO: 78
  clone 25 heavy chain

SEQ ID NO: 96 - DNA, 333 bp, Artificial Sequence
  clone 25 light chain
cagtctgtcctgacgcagccgccctcagtgtctggggccccagggcagagggtcaccatctcctgcactgggagcagctccaacatcggggcaggttatgatgtacactggtaccagcaggttccaggaacagcccccaaactcctcatctttggtagcaccgatcggccctcaggggtccctgatcgcttctctggctccaagtctggcaacacggcctccctgaccatctctgggctccaggctgaggatgaggctgattattattgccagtcctatgaccgcagcctgagtcatgtcttcggaactgggaccaaggtcaccgtcctaggc

SEQ ID NO: 97 - DNA, 375 bp, Artificial Sequence
  clone 26 heavy chain
gaggtgcagctggtggagtctgggggaggcctggccaagcctggggggtccctgagactctcctgtgcagcctctggattcaccttcactagttataggatgcattgggtccgccaggctccagggaaggggctggagtgggtctcatcaattactggtggtggtaattatatagagtacgcagactcagtgaagggccggttcaccatctccagagacaacgccaagaactcactggatctgcaaatgaacagcctgagagccgaggacacggctatttattactgtgcgagagatatgtatggtttggggagttattattcgcctaactacttcgacccctggggccagggaaccctggtcaccgtctcctca

SEQ ID NO: 98 - DNA, 333 bp, Artificial Sequence
  clone 26 light chain
cagtctgtgctgacgcagccgccctcagtgtctggggccccagggcagagggtcaccatctcctgcactgggagcagctccaacatcggggcaggttatgatgtacactggtatcagcagcttccgggagcagcccccagactcctcatgtttggtaacagcaatcggccctcgggggtacctgaccgcttctctggctccaagtctggcacctccgcctccctggccatcactggtctccaggctgaggatgaggctgattattactgccagtcctatgaccgcagcctgagtcatgtcttcggaactgggaccaaggtcaccgtcctaggc

SEQ ID NO: 99 - DNA, 375 bp, Artificial Sequence; identical to SEQ ID NO: 38
  clone 27 heavy chain

SEQ ID NO: 100 - DNA, 333 bp, Artificial Sequence
  clone 27 light chain
tcctatgagctgactcagccaccctcagtgtctggggccccagggcagagggtcaccatctcctgcactgggagcagctccaacatcggggcaggttatgatgtacactggtatcagcagcttccgggagcagcccccagactcctcatgtttggtaacagcaatcggccctcgggggtacctgaccgcttctctggctccaagtctggcacctccgcctccctggccatcactggtctccaggctgaggatgaggctgattattactgccagtcctatgacagtagcctgagttatgtcttcggaactgggaccaaggtcaccgtcctaggc

SEQ ID NO: 101 - DNA, 333 bp, Artificial Sequence
  clone 27m light chain
cagtctgtgctgacgcagccgccctcagtgtctggggccccagggcagagggtcaccatctcctgcactgggagcagctccaacatcggggcaggttatgatgtacactggtatcagcagcttccgggagcagcccccagactcctcatgtttggtaacagcaatcggccctcgggggtacctgaccgcttctctggctccaagtctggcacctccgcctccctggccatcactggtctccaggctgaggatgaggctgattattactgccagtcctatgacagtagcctgagttatgtcttcggaactgggaccaaggtcaccgtcctaggc

SEQ ID NO: 102 - DNA, 375 bp, Artificial Sequence; identical to SEQ ID NO: 78
  clone 28 heavy chain

SEQ ID NO: 103 - DNA, 333 bp, Artificial Sequence
  clone 28 light chain
cagtctgtgctgacgcagccgccctcagtgtctggggccccagggcagagggtcaccatctcctgcactgggagcagctccaacatcggggcaggttatgatgtacactggtatcagcagcttccgggagcagcccccagactcctcatgtttggtaacagcaatcggccctcgggggtacctgaccgcttctctggctccaagtctggcacctccgcctccctggccatcactggtctccaggctgaggatgaggctgattattactgccagtcctatgacagtagcctgagtcatgtcttcggaactgggaccaaggtcaccgtcctaggc

SEQ ID NO: 104 - DNA, 375 bp, Artificial Sequence
  clone 29 heavy chain
gaggtgcagctggtggagtctgggggaggcttggtccagcctggggggtccctgagactctcctgtgcagcctctggattcaccttcactagttataggatgcattgggtccgccaggctccagggaaggggctggagtgggtctcatcaattactggtggtggtaattatatagagtacgcagactcagtgaagggccggttcaccatctccagagacaacgccaagaactcactggatctgcaaatgaacagcctgagagccgaggacacggctatttattactgtgcgagagatatgtatggtttggggagttattattcgcctaactacttcgacccctggggccagggaaccctggtcaccgtctcctca

SEQ ID NO: 105 - DNA, 333 bp, Artificial Sequence; identical to SEQ ID NO: 101
  clone 29 light chain

SEQ ID NO: 106 - DNA, 357 bp, Artificial Sequence
  clone 30 heavy chain
gaggtgcagctggtggagtctgggggaggcttggtacagcctggggggtccctgagactctcctgtgcagcatctgaattcacctttagcatgaactgggtccgacaggctccagggaaggggctggagtgggtctcatcagttcgaggtggcggtactgaaacatactatgcagactccgtgaagggccggttcaccgtctccagagacaattccaagaacaccctgcatctgcaaatgaacagcctgagagccgaggacacggccctttattactgtgcgggcggccctatagtggaacccaacattgactactttaactcctggggccagggaaccctggtcaccgtctcctca

SEQ ID NO: 107 - DNA, 379 bp, Artificial Sequence
  clone 30 light chain
tgctgtgggtgagtggtacctgtgggcagtctgtgctgacgcagccgccctcagtgtctggggccccagggcagagggtcaccatctcctgcactgggagcagctccaacatcggggcaggttatgatgtacactggtaccagcagcttccaggaagagcccccaaactcctcatctttgctaacaccaatcggccctcaggggtccctgaccgattctctggctccaagtctggcgcctctgcctccctggccatcactggcctccaggctgacgatgaggctgattattactgccagtcttatgacagcaaacatcatgtggtctttggcacagggaccaagctgaccgtcctaggccaacctaaggccaatcccac

SEQ ID NO: 108 - DNA, 333 bp, Artificial Sequence
  clone 30m light chain
cagtctgtgctgacgcagccgccctcagtgtctggggccccagggcagagggtcaccatctcctgcactgggagcagctccaacatcggggcaggttatgatgtacactggtaccagcagcttccaggaagagcccccaaactcctcatctttgctaacaccaatcggccctcaggggtccctgaccgattctctggctccaagtctggcgcctctgcctccctggccatcactggcctccaggctgacgatgaggctgattattactgccagtcttatgacagcaaacatcatgtggtctttggcacagggaccaagctgaccgtcctaggc

SEQ ID NO: 109 - DNA, 384 bp, Artificial Sequence
  clone 31 heavy chain
gaggtgcagctggtggagtctgggggaggcttggtccagcctggggggtccctgagactctcctgtgcagcctctgggttctcctttaggagttattggatgagctggctccgccaggccccagggaaggggctgcagtgggtggccaacataaagccagacggaagtgtggaaagttatgtggactccgtggagggccgattcaccatctccagagacaacgccaagaattcactgtttctgcaaatgaacagcctgtcagccgaggacatggctgtttattactgtgcgaggacggacgacggcagcagctggttcgtgtccaccagtagtttctacggtatggacgtctggggccaagggaccacggtcaccgtctcctca

SEQ ID NO: 110 - DNA, 333 bp, Artificial Sequence
  clone 31 light chain
cagtctgtgttgacgcagccgccctcagtgtctggggccccagggcagagggtcaccatctcctgcactgggagcagctccaacatcggggcaggttatgatgtacactggtaccagcaggttccaggaacagcccccaaactcctcatctttggtagcaccaatcggccctcaggggtccctgaccgattctctggctccaagtctggcgcctcagcctccctggccatcattgggctccagactgaggatgaggctgattattactgccagtcctatgaccgcagcctgagtcatgtcttcggaactggcacccagctgaccgacctcggc

SEQ ID NO: 111 - DNA, 378 bp, Artificial Sequence
  clone 32 heavy chain
gaggtgcagctggtggagtctgggggaggcctggtcaagcctggggggtccctgagactctcctgtgcagcctctggattcaccttcagtagctataccatgcactgggtccgccaggctccagggaaggggctggagtgggtctcgtccataactggtggcagtagttatgtcgactactcagcctcagtgaagggccgattcaccatctcccgagacaattccaagaacacgctgtatctgcaaatgagcagcctgagaactgacgacacggccgtatatttctgtgcgaaagaccaacgtggagacagctatgactcggttatgaactggtacttcgatctctggggccgtggcaccacggtcaccgtctcctca

SEQ ID NO: 112 - DNA, 333 bp, Artificial Sequence
  clone 32 light chain
cagtctgtgttgacgcagccgccctcagtgtctggggccccagggcagagggtcaccatttcctgcactgggaacagctccaacctcggggcaggttatgatgtacactggtaccagcaggttccaggaacagcccccaaactcctcatctttggtagcaccaatcggccctcaggggtccctgaccgattctctggctccaagtctggcgcctcagcctccctgacaatctctgggctccaggctgaggacgaggctgattattactgctgttcgtatgcagctagtagctctagggtcttcggaactggcaccaaggtgaccgtcctcggc

SEQ ID NO: 113 - DNA, 426 bp, Artificial Sequence
  clone 33m heavy chain
tgctgtgggtgagtggtacctgtggggaggtgcagctggtggagtctgggggcggcctggttaagcctggggggtccctgagactctcgtgtgcagcctctgggttcaggctcagtagctatggcatgaactgggtccgccaggctccagggaaggggctggagtgggtctcatccatttctgctagtagtagttttataaactatgcagactcagtgagggaccgattcaccatctccagagacaacgccaagaactcactgtatctgcaaatgaacagcctgagagccgaggacacggctgtgtattactgtgcgagagatgattatggttcggggagttattccaactggttcgacccctggggccagggaaccctggtcaccgtctcctcagcctccaccaagggcccatcggtcttccccc

SEQ ID NO: 114 - DNA, 366 bp, Artificial Sequence
  clone 34 heavy chain
gaggtgcagctggtggagtctgggggaggcctggtcaagcctggggggtccctgagactctcctgtgcagcctctggattcaccttcagtcattatggtattagttgggtgcgccaggcccctggacaaggccttgagtggatggcctggatcagcgcttacaatggtaacacagactccatacagaaggtccagggcagagtcaccatgaccacagacacatccacgaacacagcctacttggaattgaggagcctgagatctgacgacacggccgtgtattactgtgtaagagatgtcccggccacaggaggagctgccacggctgactactggggccaaggaaccctggtcaccgtctcctca

SEQ ID NO: 115 - DNA, 423 bp, Artificial Sequence
  clone 34m heavy chain
tgctgtgggtgagtggtacctgtgggcaggttcagctggtgcagtctggagctgaggtgaagaagcctggggcctcagtgaaggtctcctgcaaggcttctggattcaccttcagtcattatggtattagttgggtgcgccaggcccctggacaaggccttgagtggatggcctggatcagcgcttacaatggtaacacagactccatacagaaggtccagggcagagtcaccatgaccacagacacatccacgaacacagcctacttggaattgaggagcctgagatctgacgacacggccgtgtattactgtgtaagagatgtcccggccacaggaggagctgccacggctgactactggggccaaggaaccctggtcaccgtctcctcagcctccaccaagggcccatcggtcttccccc

SEQ ID NO: 116 - DNA, 336 bp, Artificial Sequence
  clone 34 light chain
cagtctgtgttgacgcagccgccctcagtgtctggggccccagggcagagggtcaccatctcctgcactgggagcagctccaacatcggggcaggttatgatgtacactggtaccagcaggttccaggaacagcccccaaactcctcatctttggtagcaccaatcggccctcaggggtccctgaccgattctctggctccaagtctggcgcctcagcctccctggccatcactgggctccaggctgaggacgaggctgattattactgcagctcatatacaagcagcagcactttcgtggtatttggtggaggaacccagctgatcattttaggc

SEQ ID NO: 117 - DNA, 363 bp, Artificial Sequence
  clone 35 heavy chain
caggtgcagctggtggagtctgggggaggcgtggtccagcctgggaggtccctgagactctcctgtgcagcctctggattcaccttcaatagctatgctatgcactgggtccgccaggctccaggcaacgggctggactgggtggcaggtatatcatatgatggaggcaataaatattacgcagactccgtgaaggaccgattcaccatctcccgagacaattccaagaacacgctgtatctgcaaatgagcagcctgagaactgacgacacggctgtatattactgtgcgaaagatgccggatgggaggcttggtggtacttcgacctctggggccgtggcaccctggtcactgtctcctca

SEQ ID NO: 118 - DNA, 333 bp, Artificial Sequence
  clone 35 light chain
cagtctgccctgactcagcctgcctccgtgtctgggtctcctggacagtcgatcaccatctcctgcactggaaccagcagtgacgttggtggttataactatgtctcctggttccaacagtacccaggcaaagcccccaaactcatgatttatgatgtcagtaagcggccctcaggggtttctaatcgcttctctggctccaagtctggcaacacggcctccctgaccatctctgagctccaggctgaggatgaggctgattattactgcagctcatatacaagcagcagcactggcgtattcggcggagggaccaagctgaccgtcctaggc

SEQ ID NO: 119 - DNA, 369 bp, Artificial Sequence
  clone 36 heavy chain
gaggtgcagctggtggagtctgggggaggcttggtacagcctggggggtccctgagactctcctgtgcagcctctggaacctttaccaaatatgccatgacctgggtccgccaggctctagggaaggggctggagtgggtctcaactattggcagtggtagtgacactcactacgcagactccgtgaagggccgcttcaccatctccagagacaattccaggaacactctgtctctacaaatgaacagcctgagagccgaggacacggccgtatattactgtgccaaatatctgggaataacagtgggtgatacgggttttcggacctttgactactggggccagggaaccacggtcaccgtctcttca

SEQ ID NO: 120 - DNA, 379 bp, Artificial Sequence
  clone 36 light chain
tgctgtgggtgagtggtacctgtgggcagtctgccctgactcagcctcgctcagtgtccgggtctcctggacagtcagtcaccatctcctgcactggaaccagcagtgatgttgggagttataaccttgtctcctggtaccaacagcacccaggcaaagcccccaaactcatgatttatgatgtcagtaagcggccctcaggggtttctaatcgcttctctggctccaagtctggcaacacggcctccctgaccatctccgggctccaggctgaggatgaggctgattattactgcagctcatatgcaggcagcgggaatgtggtatttggtggaggaacccagctgatcattttaggccaacctaaggccaatcccac

SEQ ID NO: 121 - DNA, 354 bp, Artificial Sequence
  clone 37 heavy chain
caggtgcagctggtggagtctgggggaggcgtggtccagcctgggaggtccctgagactctcctgtgcagcctctggattcaccttcagtatctatgctatgcactgggtccgccaggctccaggcaaggggctagagtgggtggcagttgtttcatatgatggaagcgagaaatactacgcagactccgtgcagggccgattcaccatctccagagacaagtccaagaacaccctgtatctgcaaatgaacagcctgacagctgaggacacggctgtctattactgtgcgagagagccctgggtggggacaattggctactggggccagggaaccctggtcaccgtctcctca

SEQ ID NO: 122 - DNA, 336 bp, Artificial Sequence
  clone 37 light chain
cagtctgccctgactcagcctccctccgcgtccgggtctcctggacagtcagtcaccatctcctgcactggaaccagcagtgacgttggtggttataactatgtctcctggtaccgacagcacccaggcaaagcccccaaactcctgatttatgaggtcaataaccggccctcaggggtccctagtcgcttctctggctccaagtctggcaacacggcctccctgaccatctctgggctccaggctgaggatgaggctgattattactgcagctcatatacaagcagcagcactttcgtggtacttggtggaggaacccagctgatcattttaggc

SEQ ID NO: 123 - DNA, 372 bp, Artificial Sequence
  clone 38 heavy chain
caaatgcagctggtgcagtctgggcctgaggtgaagaagcctgggtcctcggtgaaggtctcctgcaaggcttcgggttacacctttaccgactacggtctcagctgggtccggcaggcccccggccacggccttgagtggatgggatggatcaccgcttacaatggcgacacaaactatgcacagaagttccaggacagactgtccgtgaccactgacatatccacgagcacagcctacatggaattacggagcctgaaatctgacgacacggccgtttattattgtgcgagacacgtcttttgcagtggtgatgggtgttactccggccttgggtcctggggccagggaaccctggtcaccgtctcctca

SEQ ID NO: 124 - DNA, 429 bp, Artificial Sequence
  clone 38m heavy chain
tgctgtgggtgagtggtacctgtgggcaggttcagctggtgcagtctggagctgaggtgaagaagcctggggcctcagtgaaggtctcctgcaaggcttcgggttacacctttaccgactacggtctcagctgggtccggcaggcccccggccacggccttgagtggatgggatggatcaccgcttacaatggcgacacaaactatgcacagaagttccaggacagactgtccgtgaccactgacatatccacgagcacagcctacatggaattacggagcctgaaatctgacgacacggccgtttattattgtgcgagacacgtcttttgcagtggtgatgggtgttactccggccttgggtcctggggccagggaaccctggtcaccgtctcctcagcctccaccaagggcccatcggtcttccccc

SEQ ID NO: 125 - DNA, 379 bp, Artificial Sequence
  clone 38 light chain
tgctgtgggtgagtggtacctgtgggcagtctgtgctgactcagccaccctcagcgtctgggacccccgggcagagggtcaccatctcttgttctggaagcagctccaacgtcggaagtaatactgtcaactggtaccagcagctcccaggaacggcccccaaactcctcatctacgataagaatgagcggccctcaggggtcccggaccgattctctgcctccaagtctggcacctcagcctccctggccatcagtggcctccagtctgaagatgaggctgattattactgtgcagcatgggatgacagcctgaatggttgggtgttcggtggagggaccgagctgaccgtcctaggccaacctaaggccaatcccac

SEQ ID NO: 126 - DNA, 333 bp, Artificial Sequence
  clone 38m light chain
cagtctgtgctgactcagccaccctcagcgtctggggcccccgggcagcgggtcatcatctcttgttctggaagcagctccaacgtcggaagtaatactgtcaactggtaccagcagctcccaggaacggcccccaaactcctcatctacgataagaatgagcggccctcaggggtcccggaccgattctctgcctccaagtctggcacctcagcctccctggccatcagtggcctccagtctgaagatgaggctgattattactgtgcagcatgggatgacagcctgaatggttgggtgttcggtggagggaccaagctgaccgtcctaggc

SEQ ID NO: 127 - DNA, 354 bp, Artificial Sequence
  clone 39 heavy chain
gaggtgcagctggtggagtctgggggaggcctggtcaagcctggggggtccctgagactctcctgtgcagcctctgggttcaggctcagtagctatggcatgaactgggtccgccaggctccagggaaggggctggagtgggtctcatccatttctgctagtagtagttttataaactatgcagactcagtgaggggccgattcaccatctccagagacaagtccaagaacaccctgtatctgcaaatgaacagcctgacagctgaggacacggctgtctattactgtgcgagagagccctgggtggggacaattgactactggggccagggaaccctggtcaccgtctcctca

SEQ ID NO: 128 - DNA, 336 bp, Artificial Sequence
  clone 39 light chain
cagtctgccctgactcagcctgcctccgtgtctgggtctcctggacagtcgatcaccatctcctgcactggaaccagcagtgatgttgggagttataaccttgtctcctggtaccaacagcacccaggcaaagcccccaaactcctgatttatgaggacactaagcggccctcagggatcccagaccgattctctggctccagctcaggaaacacagcttccttgaccatcactggggctcaggcggaagatgaggctgagtattactgtagttcccgggacagcagtggtaaccatctggtgttcggcggagggaccaagctgaccgtcctaggc

SEQ ID NO: 129 - DNA, 372 bp, Artificial Sequence
  clone 40 heavy chain
caggtgcagctggtgcagtctggagctgaggtgaagaagcctggggcctcagtgaaggtctcctgcaaggcttcgggttacacctttaccgactacggtctcagctgggtccggcaggcccccggccacggccttgagtggatgggatggatcaccgcttacaatggcgacacaaactatgcacagaagttccaggacagactgtccgtgaccactgacatatccacgagcacagcctacatggaattacggagcctgaaatctgacgacacggccgtttattattgtgcgagacacgtcttttgcagtggtgatgggtgttactccggccttgggtcctggggccagggaaccctggtcaccgtctcctca

SEQ ID NO: 130 - DNA, 333 bp, Artificial Sequence
  clone 40 light chain
tcctatgagctgactcagccaccctcagcgtctggggcccccgggcagcgggtcatcatctcttgttctggaagcagctccaacgtcggaagtaatactgtcaactggtaccagcagcttccaggaagagcccccaaactcctcatctttgctaacaccaatcggccctcaggggtccctgaccgattctctggctccaagtctggcacctcagcctccctggccatcagtggcctccagtctgaagatgaggctgattattactgtgcagcatgggatgacagcctgaatggttgggtgttcggtggagggaccaagctgaccgtcctaggc

SEQ ID NO: 131 - DNA, 333 bp, Artificial Sequence
  clone 40m light chain
cagtctgtgctgactcagccaccctcagcgtctggggcccccgggcagcgggtcatcatctcttgttctggaagcagctccaacgtcggaagtaatactgtcaactggtaccagcagcttccaggaagagcccccaaactcctcatctttgctaacaccaatcggccctcaggggtccctgaccgattctctggctccaagtctggcacctcagcctccctggccatcagtggcctccagtctgaagatgaggctgattattactgtgcagcatgggatgacagcctgaatggttgggtgttcggtggagggaccaagctgaccgtcctaggc

SEQ ID NO: 132 - DNA, 372 bp, Artificial Sequence
  clone 41 heavy chain
caggtgcagctggtgcagtctggggctgaggtgaagaagccgggggcctcagtgaaggtctcctgcaaggcttcgggttacacctttaccgactacggtctcagctgggtccggcaggcccccggccacggccttgagtggatgggatggatcaccgcttacaatggcgacacaaactatgcacagaagttccaggacagactgtccgtgaccactgacatatccacgagcacagcctacatggaattacggagcctgaaatctgacgacacggccgtttattattgtgcgagacacgtcttttgcagtggtgatgggtgttactccggccttgggtcctggggccagggaaccctggtcaccgtctcctca

SEQ ID NO: 133 - DNA, 333 bp, Artificial Sequence
  clone 41 light chain
tcctatgagctgactcagccactctcagcgtctgggacccccgggcagagggtcaccatctcttgttctggaagcagctccaacatcggaagtggtactgtaaactggtaccagcagctctcaggaacggcccccaaactcctcatgcatagtgataatcagcgcccctcaggggtccctgaccgattctctggctccaagtctggcacctcagcctccctggccatcagtggcctccagtctgaagatgaggctgattattactgtgcagcatgggatgacagcctgaatggttgggtgttcggtggagggaccaagctgaccgtcctaggc

SEQ ID NO: 134 - DNA, 333 bp, Artificial Sequence
  clone 41m light chain
cagtctgtgctgactcagccactctcagcgtctgggacccccgggcagagggtcaccatctcttgttctggaagcagctccaacatcggaagtggtactgtaaactggtaccagcagctctcaggaacggcccccaaactcctcatgcatagtgataatcagcgcccctcaggggtccctgaccgattctctggctccaagtctggcacctcagcctccctggccatcagtggcctccagtctgaagatgaggctgattattactgtgcagcatgggatgacagcctgaatggttgggtgttcggtggagggaccaagctgaccgtcctaggc

SEQ ID NO: 135 - DNA, 372 bp, Artificial Sequence
  clone 42 heavy chain
caggtgcagctggtgcagtctggaagtgaggtgaagaagcctggggcctcagtgaaggtctcctgcaaggcttcgggttacacctttaccgactacggtctcagctgggtccggcaggcccccggccacggccttgagtggatgggatggatcaccgcttacaatggtgacacaaactatgcacagaagttccaggacagactgtccgtgaccactgacatatccacgagcacagcctacatggaattacggagcctgaaatctgacgacacggccgtttattattgtgcgagacacgtcttttgcagtggtgatgggtgttactccggccttgggtcctggggccagggaaccctggtcaccgtctcctca

SEQ ID NO: 136 - DNA, 333 bp, Artificial Sequence
  clone 42 light chain
cagcctgtgctgactcagccaccctcagtgtctgggacccccgggcagagggtcaccatctcttgttctggaagcagctccaacatcggaagtgatactgtaaactggtaccagcagctctcaggaacggcccccaaactcctcatgcatagtgataatcagcgcccctcaggggtccctgaccgattctctggctccaagtctggcacctcagcctccctggccatcagtggcctccagtctgaagatgaggctgattattactgtgcagcatgggatgacagcctgaatggttgggtgttcggtggagggaccaagctgaccgtcctaggc

SEQ ID NO: 137 - DNA, 333 bp, Artificial Sequence
  clone 42m light chain
cagtctgtgctgactcagccaccctcagtgtctgggacccccgggcagagggtcaccatctcttgttctggaagcagctccaacatcggaagtgatactgtaaactggtaccagcagctctcaggaacggcccccaaactcctcatgcatagtgataatcagcgcccctcaggggtccctgaccgattctctggctccaagtctggcacctcagcctccctggccatcagtggcctccagtctgaagatgaggctgattattactgtgcagcatgggatgacagcctgaatggttgggtgttcggtggagggaccaagctgaccgtcctaggc

SEQ ID NO: 138 - DNA, 372 bp, Artificial Sequence
  clone 43 heavy chain
caggttcagctggtgcagtctggaagtgaggtgaagaagccgggggcctcagtgaaggtctcctgcaaggcttcgggttacacctttaccgactacggtctcagctgggtccggcaggcccccggccacggccttgagtggatgggatggatcaccgcttacaatggcgacacaaactatgcacagaagttccaggacagactgtccgtgaccactgacatatccacgagcacagcctacatggaattacggagcctgaaatctgacgacacggccgtttattattgtgcgagacacgtcttttgcagtggtgatgggtgttactccggccttgggtcctggggccagggaaccctggtcaccgtctcctca

SEQ ID NO: 139 - DNA, 333 bp, Artificial Sequence
  clone 43 light chain
cagcctgtgctgactcagccaccctcagcgtctgggacccccgggcagagggtcaccatctcttgttctggaagcagctccaacatcggaagtgatactgtaaactggtaccagcagctctcaggaacggcccccaaactcctcatgcatagtgataatcagcgcccctcaggggtccctgaccgattctctggctccaagtctggcacctcagcctccctggccatcagtggcctccagtctgaagatgaggctgattattactgtgcagcatgggatgacagcctgaatggttgggtgttcggtggagggaccaagctgaccgtcctaggc

SEQ ID NO: 140 - DNA, 333 bp, Artificial Sequence; identical to SEQ ID NO: 139
  clone 43 light chain

SEQ ID NO: 141 - DNA, 333 bp, Artificial Sequence
  clone 43m light chain
cagtctgtgctgactcagccaccctcagcgtctgggacccccgggcagagggtcaccatctcttgttctggaagcagctccaacatcggaagtgatactgtaaactggtaccagcagctctcaggaacggcccccaaactcctcatgcatagtgataatcagcgcccctcaggggtccctgaccgattctctggctccaagtctggcacctcagcctccctggccatcagtggcctccagtctgaagatgaggctgattattactgtgcagcatgggatgacagcctgaatggttgggtgttcggtggagggaccaagctgaccgtcctaggc

SEQ ID NO: 142 - DNA, 372 bp, Artificial Sequence
  clone 44 heavy chain
caggtgcagctggtgcagtctggagctgaggtgaagaagccgggggcctcagtgaaagtctcctgcaaggcttcgggttacacctttaccgactacggtctcagctgggtccggcaggcccccggccacggccttgagtggatgggatggatcaccgcttacaatggcgacacaaactatgcacagaagttccaggacagactgtccgtgaccactgacatatccacgagcacagcctacatggaattacggagcctgaaatctgacgacacggccgtttattattgtgcgagacacgtcttttgcagtggtgatgggtgttactccggccttgggtcctggggccagggaaccctggtcaccgtctcctca

SEQ ID NO: 143 - DNA, 333 bp, Artificial Sequence
  clone 44 light chain
cagtctgtgctgactcagccaccctcagcgtctgggacccccgggcagagggtcaccatctcttgttctggaagcagctccaacatcggaagtaatactgtaaactggtaccagcagctcccaggaacggcccccaaactcctcatctatagtaataatcagcggccctcaggggtccctgaccgattctctggctccacgtctggcacctcagcctccctggccatcagtggactccagtctgaagatgaggctgattattactgtgcagcatgggatgacagcctgaatggttgggtgttcggtggagggaccaagctgaccgtcctaggc

SEQ ID NO: 144 - DNA, 372 bp, Artificial Sequence
  clone 45 heavy chain
caggtgcagctggtgcagtctggaagtgaggtgaagaagcctggggcctcagtgaaggtctcctgcaaggcttcgggttacacctttaccgactacggtctcagctgggtccggcaggcccccggccacggccttgagtggatgggatggatcaccgcttacaatggcgacacaaactatgcacagaagttccaggacagactgtccgtgaccactgacatatccacgagcacagcctacatggaattacggagcctgaaatctgacgacacggccgtttattattgtgcgagacacgtcttttgcagtggtgatgggtgttactccggccttgggtcctggggccagggaaccctggtcaccgtctcctca

SEQ ID NO: 145 - DNA, 333 bp, Artificial Sequence
  clone 45 light chain
tcctatgagctgactcagccactctcagcgtctgggacccccgggcagagggtcaccatctcttgttctggaagcagctccaacatcggaagtaatactgtaaactggtaccagcagctcccaggaacggcccccaaactcctcatctatagtaataatcagcggccctcaggggtccctgaccgattctctggctccaagtctggcacctcagcctccctggccatcagtgggctccagtctgaggatgaggctgattattactgtgcagcatgggatgacagcctgaatggttgggtgttcggtggagggaccaagctgaccgtcctaggc

SEQ ID NO: 146 - DNA, 333 bp, Artificial Sequence
  clone 45m light chain
cagtctgtgctgactcagccactctcagcgtctgggacccccgggcagagggtcaccatctcttgttctggaagcagctccaacatcggaagtaatactgtaaactggtaccagcagctcccaggaacggcccccaaactcctcatctatagtaataatcagcggccctcaggggtccctgaccgattctctggctccaagtctggcacctcagcctccctggccatcagtgggctccagtctgaggatgaggctgattattactgtgcagcatgggatgacagcctgaatggttgggtgttcggtggagggaccaagctgaccgtcctaggc

SEQ ID NO: 147 - DNA, 372 bp, Artificial Sequence
  clone 46 heavy chain
caggtgcagctggtgcagtctgggcctgaggtgaagaagcctgggtcctcggtgaaggtctcctgcaaggcttcgggttacacctttaccgactacggtctcagctgggtccggcaggcccccggccacggccttgagtggatgggatggatcaccgcttacaatggcgacacaaactatgcacagaagttccaggacagactgtccgtgaccactgacatatccacgagcacagcctacatggaattacggagcctgaaatctgacgacacggccgtttattattgtgcgagacacgtcttttgcagtggtgatgggtgttactccggccttgggtcctggggccagggaaccctggtcaccgtctcctca

SEQ ID NO: 148 - DNA, 333 bp, Artificial Sequence
  clone 46 light chain
tcctatgagctgactcagccaccctcagcgtctggggcccccgggcagcgggtcatcatctcttgttctggaagcagctccaacgtcggaagtaatactgtcaactggtaccagcagctcccaggaacggcccccaaactcctcatctacgataagaatgagcggccctcaggggtcccggaccgattctctgcctccaagtctggcacctcagcctccctggccatcagtggcctccagtctgaagatgaggctgattattactgtgcagcatgggatgacagcctgaatggttgggtgttcggtggagggaccaagctgaccgtcctaggc

SEQ ID NO: 149 - DNA, 333 bp, Artificial Sequence; identical to SEQ ID NO: 126
  clone 46m light chain

SEQ ID NO: 150 - DNA, 381 bp, Artificial Sequence
  clone 47 heavy chain
caggttcagctggtgcagtctggagctgaggtgaagaagcctggggcctcagtgaaggtctcctgcaaggcttctggttacaccggttacacctttaccgactacggtctcagctgggtccggcaggcccccggccacggccttgagtggatgggatggatcaccgcttacaatggcgacacaaactatgcacagaagttccaggacagactgtccgtgaccactgacatatccacgagcacagcctacatggaattacggagcctgaaatctgacgacacggccgtttattattgtgcgagacacgtcttttgcagtggtgatgggtgttactccggccttgggtcctggggccagggaaccctggtcaccgtctcctca

SEQ ID NO: 151 - DNA, 333 bp, Artificial Sequence
  clone 47 light chain
tcctatgagctgatacagccaccctcagcgtctggggcccccgggcagcgggtcatcatctcttgttctggaagcagctccaacgtcggaagtaatactgtcaactggtaccagcagctcccaggaacggcccccaaactcctcatctacgataagaatgagcggccctcaggggtcccggaccgattctctgcctccaagtctggcacctcagcctccctggccatcagtggcctccagtctgaagatgaggctgattattactgtgcagcatgggatgacagcctgaatggttgggtgttcggtggagggaccgagctgaccgtcctaggc

SEQ ID NO: 152 - DNA, 333 bp, Artificial Sequence; identical to SEQ ID NO: 126
  clone 47m light chain

SEQ ID NO: 153 - DNA, 372 bp, Artificial Sequence
  clone 48 heavy chain
caggtgcagctggtgcagtctggagctgaggtgaagaagcctgggtcctcggtgaaggtctcctgcaaggcttcgggttacacctttaccgactacggtctcagctgggtccggcaggcccccggccacggccttgagtggatgggatggatcaccgcttacaatggcgacacaaactatgcacagaagttccaggacagactgtccgtgaccactgacatatccacgagcacagcctacatggaattacggagcctgaaatctgacgacacggccgtttattattgtgcgagacacgtcttttgcagtggtgatgggtgttactccggccttgggtcctggggccagggaaccctggtcaccgtctcctca

SEQ ID NO: 154 - DNA, 333 bp, Artificial Sequence
  clone 48 light chain
cagtctgtgctgacgcagccgccctcagtgtctggggccccagggcagagggtcaccatctcttgttctggaagcagctccaacgtcggaagtaatactgtcaactggtaccagcagctcccaggaacggcccccaaactcctcatctacgataagaatgagcggccctcaggggtcccggaccgattctctgcctccaagtctggcacctcatcctccctggccatcggtgggctccggtctgaagatgaggctgattattactgtgggacatgggatgacaacctgaatggttgggtgttcggcggagggaccaagctgaccgtcctaggc

SEQ ID NO: 155 - DNA, 372 bp, Artificial Sequence; identical to SEQ ID NO: 129
  clone 49 heavy chain

SEQ ID NO: 156 - DNA, 333 bp, Artificial Sequence
  clone 49 light chain
tcctatgagctgactcagccaccctcagcgtctggggcccccgggcagcgggtcatcatctcttgttctggaagcagctccaacgtcggaagtaatactgtcaactggtaccagcagctcccaggaacggcccccaaactcctcatctacgataagaatgagcggccctcaggggtcccggaccgattctctgcctccaagtctggcacctcatcctccctggccatcggtgggctccggtctgaagatgaggctgattattactgtgcgacatgggatgacaacctgaatggttgggtgttcggcggagggaccaagctgaccgtcctaggc

SEQ ID NO: 157 - DNA, 333 bp, Artificial Sequence
  clone 49m light chain
cagtctgtgctgactcagccaccctcagcgtctggggcccccgggcagcgggtcatcatctcttgttctggaagcagctccaacgtcggaagtaatactgtcaactggtaccagcagctcccaggaacggcccccaaactcctcatctacgataagaatgagcggccctcaggggtcccggaccgattctctgcctccaagtctggcacctcatcctccctggccatcggtgggctccggtctgaagatgaggctgattattactgtgcgacatgggatgacaacctgaatggttgggtgttcggcggagggaccaagctgaccgtcctaggc

SEQ ID NO: 158 - DNA, 372 bp, Artificial Sequence; identical to SEQ ID NO: 129
  clone 50 heavy chain

SEQ ID NO: 159 - DNA, 333 bp, Artificial Sequence
  clone 50 light chain
tcctatgagctgactcagccaccctcagcgtctggggcccccgggcagcgggtcatcatctcttgttctggaagcagctccaacgtcggaagtaatactgtcaactggtaccagcagctcccaggaacggcccccaaactcctcatctacgataagaatgagcggccctcaggggtcccggaccgattctctgcctccaagtctggcacctcatcctccctggccatcggtgggctccggtctgaagatgaggctgattattactgtgggacatgggatgacaacctgaatggttgggtgttcggcggagggaccaagctgaccgtcctaggc

SEQ ID NO: 160 - DNA, 333 bp, Artificial Sequence
  clone 50m light chain
cagtctgtgctgactcagccaccctcagcgtctggggcccccgggcagcgggtcatcatctcttgttctggaagcagctccaacgtcggaagtaatactgtcaactggtaccagcagctcccaggaacggcccccaaactcctcatctacgataagaatgagcggccctcaggggtcccggaccgattctctgcctccaagtctggcacctcatcctccctggccatcggtgggctccggtctgaagatgaggctgattattactgtgggacatgggatgacaacctgaatggttgggtgttcggcggagggaccaagctgaccgtcctaggc

SEQ ID NO: 161 - DNA, 372 bp, Artificial Sequence
  clone 51 heavy chain
gaggtgcagctggtggagtctgggactgaggtgaagaagcctggggcctcagtgaaggtctcctgcaaggcttcgggttacacctttaccgactacggtctcagctgggtccggcaggcccccggccacggccttgagtggatgggatggatcaccgcttacaatggcgacacaaactatgcacagaagttccaggacagactgtccgtgaccactgacatatccacgagcacagcctacatggaattacggagcctgaaatctgacgacacggccgtttattattgtgcgagacacgtcttttgcagtggtgatgggtgttactccggccttgggtcctggggccagggaaccctggtcactgtctcctca

SEQ ID NO: 162 - DNA, 429 bp, Artificial Sequence
  clone 51m heavy chain
tgctgtgggtgagtggtacctgtggggaggtgcagctggtgcagtctggggctgaggtgaagaagcctggggcctcagtgaaggtctcctgcaaggcttcgggttacacctttaccgactacggtctcagctgggtccggcaggcccccggccacggccttgagtggatgggatggatcaccgcttacaatggcgacacaaactatgcacagaagttccaggacagactgtccgtgaccactgacatatccacgagcacagcctacatggaattacggagcctgaaatctgacgacacggccgtttattattgtgcgagacacgtcttttgcagtggtgatgggtgttactccggccttgggtcctggggccagggaaccctggtcactgtctcctcagcctccaccaagggcccatcggtcttccccc

SEQ ID NO: 163 - DNA, 333 bp, Artificial Sequence; identical to SEQ ID NO: 160
  clone 51 light chain

SEQ ID NO: 164 - DNA, 384 bp, Artificial Sequence
  clone 52 heavy chain
caggtgcagctggtgcagtctgggggaggcttggtacagcctggagggtccctgagaatctcctgtacagcctctggattcaccttcaggaattatgaaatgaattgggtccgccaggctccagggaaggggctggagtgggttgcatacattagtagtagtggtagttccagatactacgcagactctgtgaagggccgattcaccatctccagagacaacgccaagaactcactgtttctgcaaatgaacagcctgagagccgaggacatggctgtttattactgtgcgaggacggacgacggcagcagctggttcgtgtccaccagtagtttctacggtatggacgtctggggccaagggaccacggtcaccgtctcctca

SEQ ID NO: 165 - DNA, 386 bp, Artificial Sequence
  clone 52m heavy chain
gagaggtgcagctggtggagtctgggggaggcttggtacagcctggagggtccctgagaatctcctgtacagcctctggattcaccttcaggaattatgaaatgaattgggtccgccaggctccagggaaggggctggagtgggttgcatacattagtagtagtggtagttccagatactacgcagactctgtgaagggccgattcaccatctccagagacaacgccaagaactcactgtttctgcaaatgaacagcctgagagccgaggacatggctgtttattactgtgcgaggacggacgacggcagcagctggttcgtgtccaccagtagtttctacggtatggacgtctggggccaagggaccacggtcaccgtctcctca

SEQ ID NO: 166 - DNA, 330 bp, Artificial Sequence
  clone 52 light chain
gaaattgtgctgacccagtctccaggcatccagtctttgtctccaggggaaacagccaccctctcctgcagggccagtgagagtattagcagcagttacttcgcctggtaccagcagaaacctggccaggctcccaggctcctcatctatggtgcatccagcagggcctctggcatcccagacaggttcagtggcagtgggtctgggacagacttcactctcaccatcagcagactggagcctgaagattttgcagtgtattactgtcagcagtatggtagctcacctcccatcaccttcggccaagggacacgactggagattaaacga

SEQ ID NO: 167 - DNA, 384 bp, Artificial Sequence
  clone 53 heavy chain
caggtgcagctggtgcagtctgggggaggcttggtacagcctggagggtccctgagaatctcctgtacagcctctggattcaccttcaggaattatgaaatgaattgggtccgccaggctccagggaaggggctggagtgggttgcatacattagtagtagtggtagttccagatactacgcagactctgtgaagggccgattcaccatctccagagacaacgccaagaacacgctgtatctgcaaatgagcagcctgagatctgacgacacggccgtgtattactgtgcgaggacggacgacggcagcagctggttcgtgtccaccagtagtttctacggtatggacgtctggggccaagggaccacggtcaccgtctcctca

SEQ ID NO: 168 - DNA, 386 bp, Artificial Sequence
  clone 53m heavy chain
gagaggtgcagctggtggagtctgggggaggcttggtacagcctggagggtccctgagaatctcctgtacagcctctggattcaccttcaggaattatgaaatgaattgggtccgccaggctccagggaaggggctggagtgggttgcatacattagtagtagtggtagttccagatactacgcagactctgtgaagggccgattcaccatctccagagacaacgccaagaacacgctgtatctgcaaatgagcagcctgagatctgacgacacggccgtgtattactgtgcgaggacggacgacggcagcagctggttcgtgtccaccagtagtttctacggtatggacgtctggggccaagggaccacggtcaccgtctcctca

SEQ ID NO: 169 - DNA, 330 bp, Artificial Sequence
  clone 53 light chain
gatgttgtgatgactcagtctccaggcaccctgtctttgtctccaggggaaagagccaccctctcctgcagggccagtcagagtgttagtagcagctacttagcctggtaccagcagaaacctggccaggctcccaggctcctcatctacggtgtgtccagcagggccactggcatcccagacaggttcagtggcagtgggtctgggacagacttcactctcaccatcagcagactggagcctgaagattttgcagtgtattactgtcagcagtatggtagctcacctcccatcaccttcggccaggggaccaagctggagatcaaacga

SEQ ID NO: 170 - DNA, 330 bp, Artificial Sequence
  clone 53m light chain
gagattgtgctgacccagtctccaggcaccctgtctttgtctccaggggaaagagccaccctctcctgcagggccagtcagagtgttagtagcagctacttagcctggtaccagcagaaacctggccaggctcccaggctcctcatctacggtgtgtccagcagggccactggcatcccagacaggttcagtggcagtgggtctgggacagacttcactctcaccatcagcagactggagcctgaagattttgcagtgtattactgtcagcagtatggtagctcacctcccatcaccttcggccaggggaccaagctggagatcaaacgt

SEQ ID NO: 171 - DNA, 360 bp, Artificial Sequence
  clone 54 heavy chain
gaggtgcagctggtggagtctgggggaggcttggtacagcctggggggtccctgagactctcctgtgcagcctctgaattcacctttagcatgaactgggtccgacaggctccagggaaggggctggagtgggtctcatcagttcgaggtggcggtactgaaacatactatgcagactccgtgaagggccggttcaccgtctccagagacaattccaagaacacactgtatctgcagatgaacagcctgagagtcgaggacacggccgtgtattactgtacggtgtgtgttgttatgtttcggggatggtgcaactggttcgacccctggggccagggaaccctggtcaccgtctcctca

SEQ ID NO: 172 - DNA, 324 bp, Artificial Sequence
  clone 54 light chain
gacatccagttgacccagtctccatcttccgtgtctgcatctgtaggagagagagtcaccatcactcgtcgggcgagtcagaatattgacaggtggttagcttggtatcagcagaaaccagggaaagcccctgacctcctgatctttgctgcatccagtttgcagagtggggtcccatcaaggttcagcggcagtggatctgggacagatttcactctcaccatcagcagcctgcagcctgaagattttgcaacttactattgtcaacagggtaaaactttccctcccacgttcggccaggggaccaagctggagatcaaacga

SEQ ID NO: 173 - DNA, 360 bp, Artificial Sequence
  clone 55 heavy chain
gaggtgcagctgttggagtctgggggaggcttggtacagcctggggggtccctgagactctcctgtgcagcctctgaattcacctttagcatgaactgggtccgacaggctccagggaaggggctggagtgggtctcatcagttcgaggtggcggtactgaaacatactatgcagactccgtgaagggccggttcaccgtctccagagacaattccaagaacacactgtatctgcagatgaacagcctgagagtcgaggacacggccgtgtattactgtacggtgtgtgttgttatgtttcggggatggtgcaactggttcgacccctggggccagggaaccctggtcaccgtctcctca

SEQ ID NO: 174 - DNA, 324 bp, Artificial Sequence
  clone 55m light chain
gatgttgtgatgactcagtctccatcgtccctgtctgcatccgttggggacagagtcaccatcacttgccgggcaagtcagagcctcagtagttatttaaattggtatcagcagaaaccagggaaagcccctaaactgctcatctatgctacaaccaacttgcaaagtggggtcccttcaaggttcagtggcagtggatctgggacacatttcactctcaccatcgggagtctgcaacctgaagattttgcaacttattactgtcaacagagtttccagaccccgctcactttcggcggagggaccaaggtggagatcaaacga

SEQ ID NO: 175 - DNA, 324 bp, Artificial Sequence
  clone 55m light chain
gacatccagatgacccagtctccatcgtccctgtctgcatccgttggggacagagtcaccatcacttgccgggcaagtcagagcctcagtagttatttaaattggtatcagcagaaaccagggaaagcccctaaactgctcatctatgctacaaccaacttgcaaagtggggtcccttcaaggttcagtggcagtggatctgggacacatttcactctcaccatcgggagtctgcaacctgaagattttgcaacttattactgtcaacagagtttccagaccccgctcactttcggcggagggaccaagctggagatcaaacgt

SEQ ID NO: 176 - DNA, 354 bp, Artificial Sequence
  clone 56 heavy chain
caggtgcagctggtggagtctgggggaggcgtggtccagcctgggaggtccctgagactctcctgtgcagcctctggattcaccttcattagctatgtcatgcactgggtccgccaggctccaggcaaggggctggagtgggtggcagttgtttcatatgatggaagcgagaaatactacgcagactccgtgaagggccgattcaccatctccagagacaattccaagaacacgctgtatctgcaaatgaacagcctgacagctgaggacacggctgtctattactgtgcgagagagccctgggtggggacaattgactactggggccagggaaccctggtcaccgtctcctca

SEQ ID NO: 177 - DNA, 324 bp, Artificial Sequence
  clone 56 light chain
gacatccagatgacccagtctccagccaccctgtctgcatctgtaggagacagagtcaccatcacttgccgggcaagtcagagcattaacaacaatttaaattggtatcaacagaaaccagggcaagcccctaagctcctgatctatgctgcatccactttacaaggtggggtcccatcaaggttcagcggcagtggatctgggacagaattcactctcacaatcagcagcctgcagcctgaagattttgcaacttattactgtcaacagcttaatggttaccctctcactttcggcggagggaccaaggtggagatcaaacga

SEQ ID NO: 178 - DNA, 363 bp, Artificial Sequence
  clone 57 heavy chain
gaggtgcagctgttggagtctgggggaggcttggtacagcctggggggtccctgagactctcctgtgcagcctctggattcacctttagcgactatgccatgagttgggtccgccaggctccagggaaggggctggagtgggtctcaagtattactgctaatggacttatgacatactacacagactccgtgaagggccgattcaccatctcccgagacaattccaagaacacgctgtatctgcaaatgagcagcctgagaactgacgacacggctgtatattactgtgcgaaagatgccggatgggaggcttggtggtacttcgacctctggggccgtggcaccctggtcaccgtctcctca

SEQ ID NO: 179 - DNA, 339 bp, Artificial Sequence
  clone 57 light chain
gacatccagatgacccagtctccagactccctggctgtgtctctgggcgagagggccaccatcaactgcaagtccagccagagtgttttatacagctccaacaataagaactacttagcttggtaccagcagaaaccaggacagcctcctaagatgctcatttactgggcatctatccgggaaaccggggtccctgaccgattcagtggcagcgggtctgagacagatttcactctcaccatcagcagcctgcaggctgaagatgtggcagtttattactgtcagcaatattatagtactctcactttcggcggagggaccaaggtggagatcaaacga

SEQ ID NO: 180 - DNA, 384 bp, Artificial Sequence
  clone 58 heavy chain
caggtgcagctggtgcagtctggggctgaggtgaagaagcctggggcctcagtgaaggtttcctgcaaggcatctggatacaccttcaccagctactatatgcgctggctgcgacaggcccctggacaagggcttgagtggatgggaataatcgaccctagtggtggtagcacaacctatgcacagaagttccagggcagagtcagcataaccagggacacgtccacgagcacagtctacatggagctgagcagcctgagatctgaggacacggccgtgtattactgtgcgagagggaggggcgtagtaccagctggcaacccctcaacggggggggtcggcatggacgtctggggccaagggaccacggtcaccgtctcctca

SEQ ID NO: 181 - DNA, 324 bp, Artificial Sequence
  clone 58 light chain
gagattgtgctgacccagtctccagccaccgtgtctctgtctcccggggaaagaaccatgttgtcttgcagggccagtcagaatgttagtaactacttagggtggtatcagcagagacgtggccagcctcccagactcctcatttccgatgcgtccaacagggcctctggcgtcccagccaggttcagtggaagtgggtctgggacagacttcactcttactatcaccagtcttcagcctgaagattttgcagtttatttctgtcagcaccggagcagctggcccgtcactttcggcggagggaccaaggtggagatcaaacga

SEQ ID NO: 182 - DNA, 366 bp, Artificial Sequence
  clone 59 heavy chain
caggtgcagctggtgcagtctggaagtgaggtgaagaagcctggggcctcagtgaaggtctcctgcaaggcctctggatacacctttggtcattatggtattagttgggtgcgccaggcccctggacaaggccttgagtggatggcctggatcagcgcttacaatggtaacacagactccatacagaaggtccagggcagagtcaccatgaccacagacacatccacgaacacagcctacttggaattgaggagcctgagatctgacgacacggccgtgtattactgtgtaagagatgtcccggccacaggaggagctgccacggctgactactggggccagggaaccctggtcaccgtctcctca

SEQ ID NO: 183 - DNA, 339 bp, Artificial Sequence
  clone 59 light chain
gatgttgtgatgactcagtctccactctccctgcccgtcacccttggccagccggcctccatctcctgcaggtctagtcaaagcctcgtcttcagtgatggaaacacctacttgagttggtttcaacagaggccaggccaatctccaaggcgcctaatttataaggtttctaaccgggactctggggtcccagacagattcagcgccagtgggtcaggcactgatttcacactgaaaatcagcagggtggaggctgacgatgttggggtttattactgcatgcaagttacacactggcctcggacttttggccaggggaccaagctggagatcaaacga

SEQ ID NO: 184 - DNA, 366 bp, Artificial Sequence
  clone 60 heavy chain
caggtgcagctggtgcagtctgggcctgaggtgaagaagcctgggtcctcagtgaaggtctcctgcaaggcctctggatacacctttggtcattatggtattagttgggtgcgccaggcccctggacaaggccttgagtggatggcctggatcagcgcttacaatggtaacacagactccatacagaaggtccagggcagagtcaccatgaccacagacacatccacgaacacagcctacttggaattgaggagcctgagatctgacgacacggccgtgtattactgtgtaagagatgtcccggccacaggaggagctgccacggctgactactggggccagggaaccacggtcaccgtctcctca

SEQ ID NO: 185 - DNA, 339 bp, Artificial Sequence
  clone 60 light chain
gatgttgtgatgactcagtctccactctccctgcccgtcacccttggccagccggcctccatctcctgcaggtctagtcaaagcctcgtcttcagtgatggaaacacctacttgagttggtttcaacagaggccaggccaatctccaaggcgcctaatttataaggtttctaaccgggactctggggtcccagacagattcagcgccagtgggtcaggcactgatttcacactgaaaatcagcagggtggaggctgacgatgttggggtttattactgcatgcaagttacacactggcctcggacttttggccaagggacacgactggagattaaacga

SEQ ID NO: 186 - DNA, 366 bp, Artificial Sequence
  clone 61 heavy chain
caggtgcagctggtgcagtctggaagtgaggtgaagaagcctggggcctcagtgaaggtctcctgcaaggcctctggatacacctttggtcattatggtattagttgggtgcgccaggcccctggacaaggccttgagtggatggcctggatcagcgcttacaatggtaacacagactccatacagaaggtccagggcagagtcaccatgaccacagacacatccacgaacacagcctacttggaattgaggagcctgagatctgacgacacggccgtgtattactgtgtaagagatgtcccggccacaggaggagctgccacggctgactactggggccagggaaccacggtcaccgtctcctca

SEQ ID NO: 187 - DNA, 339 bp, Artificial Sequence; identical to SEQ ID NO: 183
  clone 61 light chain

SEQ ID NO: 188 - DNA, 366 bp, Artificial Sequence
  clone 62 heavy chain
caggtacagctgcagcagtctggaagtgaggtgaagaagcctggggcctcagtgaaggtctcctgcaaggcctctggatacacctttggtcattatggtattagttgggtgcgccaggcccctggacaaggccttgagtggatggcctggatcagcgcttacaatggtaacacagactccatacagaaggtccagggcagagtcaccatgaccacagacacatccacgaacacagcctacttggaattgaggagcctgagatctgacgacacggccgtgtattactgtgtaagagatgtcccggccacaggaggagctgccacggctgactactggggccagggaaccctggtcaccgtctcctca

SEQ ID NO: 189 - DNA, 423 bp, Artificial Sequence
  clone 62m heavy chain
tgctgtgggtgagtggtacctgtgggcaggtacagctggtgcagtctggagctgaggtgaagaagcctggggcctcagtgaaggtctcctgcaaggcctctggatacacctttggtcattatggtattagttgggtgcgccaggcccctggacaaggccttgagtggatggcctggatcagcgcttacaatggtaacacagactccatacagaaggtccagggcagagtcaccatgaccacagacacatccacgaacacagcctacttggaattgaggagcctgagatctgacgacacggccgtgtattactgtgtaagagatgtcccggccacaggaggagctgccacggctgactactggggccagggaaccctggtcaccgtctcctcagcctccaccaagggcccatcggtcttccccc

SEQ ID NO: 190 - DNA, 339 bp, Artificial Sequence
  clone 62 light chain
gatgttgtgatgacacagtctccactctccttacctgtcccccttggacagccggcctccatctcctgcaggtctagtcaaagcctcgtacacagtgatggaaacacctacttgagttggtttcagcagaggccaggccaatctccaaggcgcctaatttataaggtttctgaccgggactctggggtcccagacagattcagcggcagtgggtcaggcactgatttcacactgaaaatcagcagggtggaggctgaggatgttggggtttattactgcatgcaagttacacactggcctcggacttttggccaagggacacgactggagattaaacga

SEQ ID NO: 191 - DNA, 366 bp, Artificial Sequence; identical to SEQ ID NO: 182
  clone 63 heavy chain

SEQ ID NO: 192 - DNA, 339 bp, Artificial Sequence
  clone 63 light chain
gatgttgtgatgactcagtctccactctccctgcccgtcacccttggacaaccggcctccatctcctgcaagtctagtcgaagcctcgtacacagtgatggaaacacctacttgagttggtttcaacagaggccaggccaatctccaaggcgcctaatttataaggtttctaaccgggactctggggtcccagacagattcagcgccagtgggtcaggcactgatttcacactgaaaatcagcagggtggaggctgacgatgttggggtttattactgcatgcaagttacacactggcctcggacttttggccaggggaccaagctggagatcaaacga

SEQ ID NO: 193 - protein, 123 aa, Artificial Sequence
  clone 1 heavy chain
EVQLVESGGGLVKPGGSLRLSCAASGFTFSSYTMHWVRQAPGKGLEWVSSITGGSSYVDYSASVKGRFTISRDNAQSSLYLQMNSLRAEDTAVYYCARDDYGSGSYSNWFDPWGQGTLVTVSS

SEQ ID NO: 194 - protein, 111 aa, Artificial Sequence
  clone 1 light chain
QSVLTQPPSVSGAPGQRVTISCTGSSSNIGAGYDVHWYQQVPGTAPKLLIFGSTNRPSGVPDRFSGSKSGTSASLAITGLQADDEADYYCQSYDRSLSHVFGTGTKVTVLG

SEQ ID NO: 195 - protein, 123 aa, Artificial Sequence
  clone 2 heavy chain
EVQLVESGGGVVQSGRSLRLSCAGSGFTFSSYTMHWVRQAPGKGLEWVSSITGGSSYVDYSASVKGRFTISRDNAQSSLYLQMNSLRAEDTAVYYCARDDYGSGSYSNWFDPWGQGTLVTVSS

SEQ ID NO: 196 - protein, 111 aa, Artificial Sequence; identical to SEQ ID NO: 33
  clone 2 light chain

SEQ ID NO: 197 - protein, 123 aa, Artificial Sequence; identical to SEQ ID NO: 29
  clone 3 heavy chain

SEQ ID NO: 198 - protein, 111 aa, Artificial Sequence
  clone 3 light chain
QSVLTQPPSVSGAPGQRVTISCTGSSSNIGAGYDVHWYQQVPGTAPKLLIFGSTNRPSGVPDRFSGSKSGASASLAITGLQADDEADYYCQPYDRSLSHVFGTGTKVTVLR

SEQ ID NO: 199 - protein, 123 aa, Artificial Sequence; identical to SEQ ID NO: 29
  clone 4 heavy chain

SEQ ID NO: 200 - protein, 111 aa, Artificial Sequence
  clone 4 light chain
QSVLTQPPSVSGAPGQRVTISCTGSSSNIGAGYDVHWYQQVPGTAPKLLIFGSTNRPSGVPDRFSGSKSGASASLAITGLQADDEADYYCQSYDRSLSHVFGTGTKVTVLG

SEQ ID NO: 201 - protein, 123 aa, Artificial Sequence; identical to SEQ ID NO: 29
  clone 5 heavy chain

SEQ ID NO: 202 - protein, 111 aa, Artificial Sequence
  clone 5 light chain
QSVLTQPPSVSGAPGQRVTISCTGSSSNIGAGYDVHWYQQLPGAAPRLLMFGNSNRPSGVPDRFSGSKSGTSASLAITGLQAEDEADYYCQSYDRSLSHVFGTGTKVTVLG

SEQ ID NO: 203 - protein, 111 aa, Artificial Sequence
  clone 6 light chain
SYELTQPPSASGTPGQRVTISCTGSSSNIGAGYDVHWYQQLPGAAPRLLMFGNSNRPSGVPDRFSGSKSGTSASLAITGLQADDEADYYCQSYDRSLSHVFGTGTKVTVLG

SEQ ID NO: 204 - protein, 123 aa, Artificial Sequence
  clone 7 heavy chain
QVQLVQSGGGLIQPGGSLRLSCAGSGFTFSSYTMHWVRQAPGKGLEWVSSITGGSSYVDYSASVKGRFTISRDNAQSSLYLQMNSLRAEDTAVYYCARDDYGSGSYSNWFDPWGQGTLVTVSS

SEQ ID NO: 205 - protein, 111 aa, Artificial Sequence
  clone 7 light chain
QSVLTQPPSVSGAPGQRVTISCTGSSSNIGAGYDVHWYQQLPGTAPKLLIFANTNRPSGVPDRFSGSKSGASASLAITGLQADDEADYYCQSYDRSLSHVFGTGTKVTVLG

SEQ ID NO: 206 - protein, 123 aa, Artificial Sequence
  clone 8m heavy chain
EVQLVESGGGVVQSGRSLRLSCAASGFTFSSYTMHWVRQAPGKGLEWVSSITGGSSYVDYSASVKGRFTISRDNAQSSLYLQMNSLRAEDTAVYYCARDDYGSGSYSNWFDPWGQGTLVTVSS

SEQ ID NO: 207 - protein, 123 aa, Artificial Sequence; identical to SEQ ID NO: 29
  clone 10 heavy chain

SEQ ID NO: 208 - protein, 111 aa, Artificial Sequence
  clone 10 light chain
QSVLTQPPSVSGAPGQRVTISCTGNSSNLGAGYDVHWYQQLPGTAPKLLIYANTNRPSGVPDRFSGSKSGASASLAITGLQTEDEADYYCQSYDRSLSHVFGTGTKVTVLG

SEQ ID NO: 209 - protein, 111 aa, Artificial Sequence
  clone 11 light chain
QTVVTQEPSVSGAPGQRVTISCTGSSSNIGAGYDVHWYQQLPGRAPKLLIFANTNRPSGVPDRFSGSKSGASASLAITGLQADDEADYYCQSYDRSLSHVFGTGTKVTVLG

SEQ ID NO: 210 - protein, 111 aa, Artificial Sequence
  clone 12 light chain
QPVLTQPPSVSGAPGQRVTISCTGSSSNIGAGYDVHWYQQVPGTAPKLLIFGSTNRPSGVPDRFSGSKSGASASLAITGLQTEDEADYYCQSYDRSLSHVFGTGTKVTVLG

SEQ ID NO: 211 - protein, 123 aa, Artificial Sequence
  clone 14 heavy chain
QVTLKESGGGLVKPGGSLRLSCAGSGFTFSSYTMHWVRQAPGKGLEWVSSITGGSSYVDYSASVKGRFTISRDNAKNSLFLQMNSLRAEDTAVYYCARDDYGSGSYSNWFDPWGQGTLVTVSS

SEQ ID NO: 212 - protein, 111 aa, Artificial Sequence; identical to SEQ ID NO: 24
  clone 14 light chain

SEQ ID NO: 213 - protein, 125 aa, Artificial Sequence
  clone 15 heavy chain
EVQLVESGGGVVQPGRSLRLACAASGFTFNSYAMHWVRQAPGKGLEWVSSITGGSSYVDYSASVKGRFTISRDNAQSSLYLQMNSLRAEDTAVYYCARDMYGLGSYYSPNYFDPWGQGTLVTVSS

SEQ ID NO: 214 - protein, 111 aa, Artificial Sequence
  clone 15 light chain
SYELTQPPSVSGAPGQRVTISCTGSSSNIGAGYDVHWYQQLPGRAPKLLIFANTNRPSGVPDRFSGSKSGTSASLAITGLQAEDEADYYCQSYDSSLSYVFGTGTKVTVLG

SEQ ID NO: 215 - protein, 111 aa, Artificial Sequence
  clone 15m light chain
QSVLTQPPSVSGAPGQRVTISCTGSSSNIGAGYDVHWYQQLPGRAPKLLIFANTNRPSGVPDRFSGSKSGTSASLAITGLQAEDEADYYCQSYDSSLSYVFGTGTKVTVLG

SEQ ID NO: 216 - protein, 111 aa, Artificial Sequence
  clone 16m light chain
QSVLTQPLSASGTPGQRVTISCTGSSSNIGAGYDVHWYQQLPGRAPKLLIFANTNRPSGVPDRFSGSKSGTSASLAITGLQAEDEADYYCQSYDRSLSHVFGTGTKVTVLG

SEQ ID NO: 217 - protein, 123 aa, Artificial Sequence
  clone 17 heavy chain
EVQLVESGGGLVQPGGSLRLACAASGFTFSSYTMHWVRQAPGKGLEWVSSITGGSSYVDYSASVKGRFTISRDNAQSSLYLQMNSLRAEDTAVYYCARDDYGSGSYSNWFDPWGQGTLVTVSS

SEQ ID NO: 218 - protein, 111 aa, Artificial Sequence
  clone 17 light chain
SYELTQPPSVSGAPGQRVTISCTGSSSNIGAGYDVHWYQQLPGRAPKLLIFANTNRPSGVPDRFSGSKSGASASLAITGLQAEDEADYYCQSYDRSLSHVFGTGTKVTVLG

SEQ ID NO: 219 - protein, 111 aa, Artificial Sequence
  clone 17m light chain
QSVLTQPPSVSGAPGQRVTISCTGSSSNIGAGYDVHWYQQLPGRAPKLLIFANTNRPSGVPDRFSGSKSGASASLAITGLQAEDEADYYCQSYDRSLSHVFGTGTKVTVLG

SEQ ID NO: 220 - protein, 125 aa, Artificial Sequence
  clone 18 heavy chain
QVTLKESGGGLVKPGGSLRLSCAASGFTFTSYRMHWVRQAPGKGLEWVSSITGGGNYIEYADSVKGRFTISRDNAKNSLDLQMNSLRAEDTAIYYCARDMYGLGSYYSPNYFDPWGQGTLVTVSS

SEQ ID NO: 221 - protein, 111 aa, Artificial Sequence
  clone 18 light chain
SYELTQPLSVSGAPGQRVTISCTGSSSNIGAGYDVHWYQQVPGTAPKLLIFGSTNRPSGVPDRFSGSKSGASASLAITGLQADDEADYYCQSYDRSLSHVFGTGTKVTVLG

SEQ ID NO: 222 - protein, 111 aa, Artificial Sequence
  clone 18m light chain
QSVLTQPLSVSGAPGQRVTISCTGSSSNIGAGYDVHWYQQVPGTAPKLLIFGSTNRPSGVPDRFSGSKSGASASLAITGLQADDEADYYCQSYDRSLSHVFGTGTKVTVLG

SEQ ID NO: 223 - protein, 125 aa, Artificial Sequence
  clone 19 heavy chain
EVQLVESGGGLVKPGGSLRLSCAASGFTFTSYRMHWVRQAPGKRLEWVSSITGGGNYIEYADSVKGRFTISRDNAKNSLDLQMNSLRAEDTAIYYCARDMYGLGSYYSPNYFDPWGQGTLVTVSS

SEQ ID NO: 224 - protein, 111 aa, Artificial Sequence; identical to SEQ ID NO: 33
  clone 19 light chain

SEQ ID NO: 225 - protein, 125 aa, Artificial Sequence
  clone 20 heavy chain
EVQLVESGGGLVKPGGSLRLSCAASGFTFTSYRMHWVRQAPGKGLEWVSSITGGGNYIEYADSVKGRFTISRDNAKNSLDLQMNSLRAEDTAIYYCARDMYGLGSYYSPNYFDPWGQGTLVTVSS

SEQ ID NO: 226 - protein, 111 aa, Artificial Sequence; identical to SEQ ID NO: 210
  clone 20 light chain

SEQ ID NO: 227 - protein, 111 aa, Artificial Sequence; identical to SEQ ID NO: 33
  clone 20m light chain

SEQ ID NO: 228 - protein, 125 aa, Artificial Sequence; identical to SEQ ID NO: 220
  clone 21 heavy chain

SEQ ID NO: 229 - protein, 111 aa, Artificial Sequence
  clone 21 light chain
QSVLTQPPSVSGAPGQRVTISCTGSSSNIGAGYDVHWYQQLPGTAPKLLIFGSTNRPSGVPDRFSGSKSGASASLAITGLQTEDEADYYCQSYDRSLSHVFGTGTKVTVLG

SEQ ID NO: 230 - protein, 125 aa, Artificial Sequence; identical to SEQ ID NO: 225
  clone 22 heavy chain

SEQ ID NO: 231 - protein, 111 aa, Artificial Sequence; identical to SEQ ID NO: 24
  clone 22 light chain

SEQ ID NO: 232 - protein, 125 aa, Artificial Sequence
  clone 23 heavy chain
QVQLVQSGGGLVKPGGSLRLSCAASGFTFTSYRMHWVRQAPGKGLEWVSSITGGGNYIEYADSVKGRFTISRDNAKNSLDLQMNSLRAEDTAIYYCARDMYGLGSYYSPNYFDPWGQGTTVTVSS

SEQ ID NO: 233 - protein, 111 aa, Artificial Sequence
  clone 23 light chain
QSVLTQPPSVSGAPGQRVTISCTGSSSNIGAGYDVHWYQQLPGRAPKLLIFANTNRPSGVPDRFSGSKSGASASLAISGLQAEDEAHYYCQSYDRSLNVVFGGGTELTVLG

SEQ ID NO: 234 - protein, 125 aa, Artificial Sequence; identical to SEQ ID NO: 225
  clone 24 heavy chain

SEQ ID NO: 235 - protein, 112 aa, Artificial Sequence
  clone 24 light chain
QSVLTQPPSVSGAPGQRVTISCTGSSSNIGAGYDVHWYQQVPGTAPKLLIFGSTNRPSGVPDRFSGSKSGASASLAITGLQTEDEADYYCQSYDRSLSAWVFGGGTKLTVLG

SEQ ID NO: 236 - protein, 125 aa, Artificial Sequence; identical to SEQ ID NO: 225
  clone 25 heavy chain

SEQ ID NO: 237 - protein, 111 aa, Artificial Sequence
  clone 25 light chain
QSVLTQPPSVSGAPGQRVTISCTGSSSNIGAGYDVHWYQQVPGTAPKLLIFGSTDRPSGVPDRFSGSKSGNTASLTISGLQAEDEADYYCQSYDRSLSHVFGTGTKVTVLG

SEQ ID NO: 238 - protein, 125 aa, Artificial Sequence
  clone 26 heavy chain
EVQLVESGGGLAKPGGSLRLSCAASGFTFTSYRMHWVRQAPGKGLEWVSSITGGGNYIEYADSVKGRFTISRDNAKNSLDLQMNSLRAEDTAIYYCARDMYGLGSYYSPNYFDPWGQGTLVTVSS

SEQ ID NO: 239 - protein, 111 aa, Artificial Sequence; identical to SEQ ID NO: 202
  clone 26 light chain

SEQ ID NO: 240 - protein, 125 aa, Artificial Sequence; identical to SEQ ID NO: 23
  clone 27 heavy chain

SEQ ID NO: 241 - protein, 111 aa, Artificial Sequence
  clone 27 light chain
SYELTQPPSVSGAPGQRVTISCTGSSSNIGAGYDVHWYQQLPGAAPRLLMFGNSNRPSGVPDRFSGSKSGTSASLAITGLQAEDEADYYCQSYDSSLSYVFGTGTKVTVLG

SEQ ID NO: 242 - protein, 111 aa, Artificial Sequence
  clone 27m light chain
QSVLTQPPSVSGAPGQRVTISCTGSSSNIGAGYDVHWYQQLPGAAPRLLMFGNSNRPSGVPDRFSGSKSGTSASLAITGLQAEDEADYYCQSYDSSLSYVFGTGTKVTVLG

SEQ ID NO: 243 - protein, 125 aa, Artificial Sequence; identical to SEQ ID NO: 225
  clone 28 heavy chain

SEQ ID NO: 244 - protein, 111 aa, Artificial Sequence
  clone 28 light chain
QSVLTQPPSVSGAPGQRVTISCTGSSSNIGAGYDVHWYQQLPGAAPRLLMFGNSNRPSGVPDRFSGSKSGTSASLAITGLQAEDEADYYCQSYDSSLSHVFGTGTKVTVLG

SEQ ID NO: 245 - protein, 125 aa, Artificial Sequence
  clone 29 heavy chain
EVQLVESGGGLVQPGGSLRLSCAASGFTFTSYRMHWVRQAPGKGLEWVSSITGGGNYIEYADSVKGRFTISRDNAKNSLDLQMNSLRAEDTAIYYCARDMYGLGSYYSPNYFDPWGQGTLVTVSS

SEQ ID NO: 246 - protein, 111 aa, Artificial Sequence; identical to SEQ ID NO: 242
  clone 29 light chain

SEQ ID NO: 247 - protein, 119 aa, Artificial Sequence
  clone 30 heavy chain
EVQLVESGGGLVQPGGSLRLSCAASEFTFSMNWVRQAPGKGLEWVSSVRGGGTETYYADSVKGRFTVSRDNSKNTLHLQMNSLRAEDTALYYCAGGPIVEPNIDYFNSWGQGTLVTVSS

SEQ ID NO: 248 - protein, 111 aa, Artificial Sequence
  clone 30 light chain
QSVLTQPPSVSGAPGQRVTISCTGSSSNIGAGYDVHWYQQLPGRAPKLLIFANTNRPSGVPDRFSGSKSGASASLAITGLQADDEADYYCQSYDSKHHVVFGTGTKLTVLG

SEQ ID NO: 249 - protein, 111 aa, Artificial Sequence; identical to SEQ ID NO: 248
  clone 30m light chain

SEQ ID NO: 250 - protein, 128 aa, Artificial Sequence
  clone 31 heavy chain
EVQLVESGGGLVQPGGSLRLSCAASGFSFRSYWMSWLRQAPGKGLQWVANIKPDGSVESYVDSVEGRFTISRDNAKNSLFLQMNSLSAEDMAVYYCARTDDGSSWFVSTSSFYGMDVWGQGTTVTVSS

SEQ ID NO: 251 - protein, 111 aa, Artificial Sequence
  clone 31 light chain
QSVLTQPPSVSGAPGQRVTISCTGSSSNIGAGYDVHWYQQVPGTAPKLLIFGSTNRPSGVPDRFSGSKSGASASLAIIGLQTEDEADYYCQSYDRSLSHVFGTGTQLTDLG

SEQ ID NO: 252 - protein, 126 aa, Artificial Sequence
  clone 32 heavy chain
EVQLVESGGGLVKPGGSLRLSCAASGFTFSSYTMHWVRQAPGKGLEWVSSITGGSSYVDYSASVKGRFTISRDNSKNTLYLQMSSLRTDDTAVYFCAKDQRGDSYDSVMNWYFDLWGRGTTVTVSS

SEQ ID NO: 253 - protein, 111 aa, Artificial Sequence
  clone 32 light chain
QSVLTQPPSVSGAPGQRVTISCTGNSSNLGAGYDVHWYQQVPGTAPKLLIFGSTNRPSGVPDRFSGSKSGASASLTISGLQAEDEADYYCCSYAASSSRVFGTGTKVTVLG

SEQ ID NO: 254 - protein, 123 aa, Artificial Sequence
  clone 33m heavy chain
EVQLVESGGGLVKPGGSLRLSCAASGFRLSSYGMNWVRQAPGKGLEWVSSISASSSFINYADSVRDRFTISRDNAKNSLYLQMNSLRAEDTAVYYCARDDYGSGSYSNWFDPWGQGTLVTVSS

SEQ ID NO: 255 - protein, 122 aa, Artificial Sequence
  clone 34 heavy chain
EVQLVESGGGLVKPGGSLRLSCAASGFTFSHYGISWVRQAPGQGLEWMAWISAYNGNTDSIQKVQGRVTMTTDTSTNTAYLELRSLRSDDTAVYYCVRDVPATGGAATADYWGQGTLVTVSS

SEQ ID NO: 256 - protein, 122 aa, Artificial Sequence
  clone 34m heavy chain
QVQLVQSGAEVKKPGASVKVSCKASGFTFSHYGISWVRQAPGQGLEWMAWISAYNGNTDSIQKVQGRVTMTTDTSTNTAYLELRSLRSDDTAVYYCVRDVPATGGAATADYWGQGTLVTVSS

SEQ ID NO: 257 - protein, 112 aa, Artificial Sequence
  clone 34 light chain
QSVLTQPPSVSGAPGQRVTISCTGSSSNIGAGYDVHWYQQVPGTAPKLLIFGSTNRPSGVPDRFSGSKSGASASLAITGLQAEDEADYYCSSYTSSSTFVVFGGGTQLIILG

SEQ ID NO: 258 - protein, 121 aa, Artificial Sequence
  clone 35 heavy chain
QVQLVESGGGVVQPGRSLRLSCAASGFTFNSYAMHWVRQAPGNGLDWVAGISYDGGNKYYADSVKDRFTISRDNSKNTLYLQMSSLRTDDTAVYYCAKDAGWEAWWYFDLWGRGTLVTVSS

SEQ ID NO: 259 - protein, 111 aa, Artificial Sequence
  clone 35 light chain
QSALTQPASVSGSPGQSITISCTGTSSDVGGYNYVSWFQQYPGKAPKLMIYDVSKRPSGVSNRFSGSKSGNTASLTISELQAEDEADYYCSSYTSSSTGVFGGGTKLTVLG

SEQ ID NO: 260 - protein, 123 aa, Artificial Sequence
  clone 36 heavy chain
EVQLVESGGGLVQPGGSLRLSCAASGTFTKYAMTWVRQALGKGLEWVSTIGSGSDTHYADSVKGRFTISRDNSRNTLSLQMNSLRAEDTAVYYCAKYLGITVGDTGFRTFDYWGQGTTVTVSS

SEQ ID NO: 261 - protein, 111 aa, Artificial Sequence
  clone 36 light chain
QSALTQPRSVSGSPGQSVTISCTGTSSDVGSYNLVSWYQQHPGKAPKLMIYDVSKRPSGVSNRFSGSKSGNTASLTISGLQAEDEADYYCSSYAGSGNVVFGGGTQLIILG

SEQ ID NO: 262 - protein, 118 aa, Artificial Sequence
  clone 37 heavy chain
QVQLVESGGGVVQPGRSLRLSCAASGFTFSIYAMHWVRQAPGKGLEWVAVVSYDGSEKYYADSVQGRFTISRDKSKNTLYLQMNSLTAEDTAVYYCAREPWVGTIGYWGQGTLVTVSS

SEQ ID NO: 263 - protein, 112 aa, Artificial Sequence
  clone 37 light chain
QSALTQPPSASGSPGQSVTISCTGTSSDVGGYNYVSWYRQHPGKAPKLLIYEVNNRPSGVPSRFSGSKSGNTASLTISGLQAEDEADYYCSSYTSSSTFVVLGGGTQLIILG

SEQ ID NO: 264 - protein, 124 aa, Artificial Sequence
  clone 38 heavy chain
QMQLVQSGPEVKKPGSSVKVSCKASGYTFTDYGLSWVRQAPGHGLEWMGWITAYNGDTNYAQKFQDRLSVTTDISTSTAYMELRSLKSDDTAVYYCARHVFCSGDGCYSGLGSWGQGTLVTVSS

SEQ ID NO: 265 - protein, 124 aa, Artificial Sequence
  clone 38m heavy chain
QVQLVQSGAEVKKPGASVKVSCKASGYTFTDYGLSWVRQAPGHGLEWMGWITAYNGDTNYAQKFQDRLSVTTDISTSTAYMELRSLKSDDTAVYYCARHVFCSGDGCYSGLGSWGQGTLVTVSS

SEQ ID NO: 266 - protein, 111 aa, Artificial Sequence
  clone 38 light chain
QSVLTQPPSASGTPGQRVTISCSGSSSNVGSNTVNWYQQLPGTAPKLLIYDKNERPSGVPDRFSASKSGTSASLAISGLQSEDEADYYCAAWDDSLNGWVFGGGTELTVLG

SEQ ID NO: 267 - protein, 111 aa, Artificial Sequence
  clone 38m light chain
QSVLTQPPSASGAPGQRVIISCSGSSSNVGSNTVNWYQQLPGTAPKLLIYDKNERPSGVPDRFSASKSGTSASLAISGLQSEDEADYYCAAWDDSLNGWVFGGGTKLTVLG

SEQ ID NO: 268 - protein, 118 aa, Artificial Sequence
  clone 39 heavy chain
EVQLVESGGGLVKPGGSLRLSCAASGFRLSSYGMNWVRQAPGKGLEWVSSISASSSFINYADSVRGRFTISRDKSKNTLYLQMNSLTAEDTAVYYCAREPWVGTIDYWGQGTLVTVSS

SEQ ID NO: 269 - protein, 112 aa, Artificial Sequence
  clone 39 light chain
QSALTQPASVSGSPGQSITISCTGTSSDVGSYNLVSWYQQHPGKAPKLLIYEDTKRPSGIPDRFSGSSSGNTASLTITGAQAEDEAEYYCSSRDSSGNHLVFGGGTKLTVLG

SEQ ID NO: 270 - protein, 124 aa, Artificial Sequence; identical to SEQ ID NO: 265
  clone 40 heavy chain

SEQ ID NO: 271 - protein, 111 aa, Artificial Sequence
  clone 40 light chain
SYELTQPPSASGAPGQRVIISCSGSSSNVGSNTVNWYQQLPGRAPKLLIFANTNRPSGVPDRFSGSKSGTSASLAISGLQSEDEADYYCAAWDDSLNGWVFGGGTKLTVLG

SEQ ID NO: 272 - protein, 111 aa, Artificial Sequence
  clone 40m light chain
QSVLTQPPSASGAPGQRVIISCSGSSSNVGSNTVNWYQQLPGRAPKLLIFANTNRPSGVPDRFSGSKSGTSASLAISGLQSEDEADYYCAAWDDSLNGWVFGGGTKLTVLG

SEQ ID NO: 273 - protein, 124 aa, Artificial Sequence; identical to SEQ ID NO: 265
  clone 41 heavy chain

SEQ ID NO: 274 - protein, 111 aa, Artificial Sequence
  clone 41 light chain
SYELTQPLSASGTPGQRVTISCSGSSSNIGSGTVNWYQQLSGTAPKLLMHSDNQRPSGVPDRFSGSKSGTSASLAISGLQSEDEADYYCAAWDDSLNGWVFGGGTKLTVLG

SEQ ID NO: 275 - protein, 111 aa, Artificial Sequence
  clone 41m light chain
QSVLTQPLSASGTPGQRVTISCSGSSSNIGSGTVNWYQQLSGTAPKLLMHSDNQRPSGVPDRFSGSKSGTSASLAISGLQSEDEADYYCAAWDDSLNGWVFGGGTKLTVLG

SEQ ID NO: 276 - protein, 124 aa, Artificial Sequence
  clone 42 heavy chain
QVQLVQSGSEVKKPGASVKVSCKASGYTFTDYGLSWVRQAPGHGLEWMGWITAYNGDTNYAQKFQDRLSVTTDISTSTAYMELRSLKSDDTAVYYCARHVFCSGDGCYSGLGSWGQGTLVTVSS

SEQ ID NO: 277 - protein, 111 aa, Artificial Sequence
  clone 42 light chain
QPVLTQPPSVSGTPGQRVTISCSGSSSNIGSDTVNWYQQLSGTAPKLLMHSDNQRPSGVPDRFSGSKSGTSASLAISGLQSEDEADYYCAAWDDSLNGWVFGGGTKLTVLG

SEQ ID NO: 278 - protein, 111 aa, Artificial Sequence
  clone 42m light chain
QSVLTQPPSVSGTPGQRVTISCSGSSSNIGSDTVNWYQQLSGTAPKLLMHSDNQRPSGVPDRFSGSKSGTSASLAISGLQSEDEADYYCAAWDDSLNGWVFGGGTKLTVLG

SEQ ID NO: 279 - protein, 124 aa, Artificial Sequence; identical to SEQ ID NO: 276
  clone 43 heavy chain

SEQ ID NO: 280 - protein, 124 aa, Artificial Sequence; identical to SEQ ID NO: 276
  clone 43m heavy chain

SEQ ID NO: 281 - protein, 111 aa, Artificial Sequence
  clone 43 light chain
QPVLTQPPSASGTPGQRVTISCSGSSSNIGSDTVNWYQQLSGTAPKLLMHSDNQRPSGVPDRFSGSKSGTSASLAISGLQSEDEADYYCAAWDDSLNGWVFGGGTKLTVLG

SEQ ID NO: 282 - protein, 111 aa, Artificial Sequence
  clone 43m light chain
QSVLTQPPSASGTPGQRVTISCSGSSSNIGSDTVNWYQQLSGTAPKLLMHSDNQRPSGVPDRFSGSKSGTSASLAISGLQSEDEADYYCAAWDDSLNGWVFGGGTKLTVLG

SEQ ID NO: 283 - protein, 124 aa, Artificial Sequence; identical to SEQ ID NO: 265
  clone 44 heavy chain

SEQ ID NO: 284 - protein, 111 aa, Artificial Sequence
  clone 44 light chain
QSVLTQPPSASGTPGQRVTISCSGSSSNIGSNTVNWYQQLPGTAPKLLIYSNNQRPSGVPDRFSGSTSGTSASLAISGLQSEDEADYYCAAWDDSLNGWVFGGGTKLTVLG

SEQ ID NO: 285 - protein, 124 aa, Artificial Sequence; identical to SEQ ID NO: 276
  clone 45 heavy chain

SEQ ID NO: 286 - protein, 111 aa, Artificial Sequence
  clone 45 light chain
SYELTQPLSASGTPGQRVTISCSGSSSNIGSNTVNWYQQLPGTAPKLLIYSNNQRPSGVPDRFSGSKSGTSASLAISGLQSEDEADYYCAAWDDSLNGWVFGGGTKLTVLG

SEQ ID NO: 287 - protein, 111 aa, Artificial Sequence
  clone 45m light chain
QSVLTQPLSASGTPGQRVTISCSGSSSNIGSNTVNWYQQLPGTAPKLLIYSNNQRPSGVPDRFSGSKSGTSASLAISGLQSEDEADYYCAAWDDSLNGWVFGGGTKLTVLG

SEQ ID NO: 288 - protein, 124 aa, Artificial Sequence
  clone 46 heavy chain
QVQLVQSGPEVKKPGSSVKVSCKASGYTFTDYGLSWVRQAPGHGLEWMGWITAYNGDTNYAQKFQDRLSVTTDISTSTAYMELRSLKSDDTAVYYCARHVFCSGDGCYSGLGSWGQGTLVTVSS

SEQ ID NO: 289 - protein, 111 aa, Artificial Sequence
  clone 46 light chain
SYELTQPPSASGAPGQRVIISCSGSSSNVGSNTVNWYQQLPGTAPKLLIYDKNERPSGVPDRFSASKSGTSASLAISGLQSEDEADYYCAAWDDSLNGWVFGGGTKLTVLG

SEQ ID NO: 290 - protein, 111 aa, Artificial Sequence; identical to SEQ ID NO: 267
  clone 46m light chain

SEQ ID NO: 291 - protein, 127 aa, Artificial Sequence
  clone 47 heavy chain
QVQLVQSGAEVKKPGASVKVSCKASGYTGYTFTDYGLSWVRQAPGHGLEWMGWITAYNGDTNYAQKFQDRLSVTTDISTSTAYMELRSLKSDDTAVYYCARHVFCSGDGCYSGLGSWGQGTLVTVSS

SEQ ID NO: 292 - protein, 111 aa, Artificial Sequence
  clone 47 light chain
SYELIQPPSASGAPGQRVIISCSGSSSNVGSNTVNWYQQLPGTAPKLLIYDKNERPSGVPDRFSASKSGTSASLAISGLQSEDEADYYCAAWDDSLNGWVFGGGTELTVLG

SEQ ID NO: 293 - protein, 111 aa, Artificial Sequence; identical to SEQ ID NO: 267
  clone 47m light chain

SEQ ID NO: 294 - protein, 124 aa, Artificial Sequence
  clone 48 heavy chain
QVQLVQSGAEVKKPGSSVKVSCKASGYTFTDYGLSWVRQAPGHGLEWMGWITAYNGDTNYAQKFQDRLSVTTDISTSTAYMELRSLKSDDTAVYYCARHVFCSGDGCYSGLGSWGQGTLVTVSS

SEQ ID NO: 295 - protein, 111 aa, Artificial Sequence
  clone 48 light chain
QSVLTQPPSVSGAPGQRVTISCSGSSSNVGSNTVNWYQQLPGTAPKLLIYDKNERPSGVPDRFSASKSGTSSSLAIGGLRSEDEADYYCGTWDDNLNGWVFGGGTKLTVLG

SEQ ID NO: 296 - protein, 124 aa, Artificial Sequence; identical to SEQ ID NO: 265
  clone 49 heavy chain

SEQ ID NO: 297 - protein, 111 aa, Artificial Sequence
  clone 49 light chain
SYELTQPPSASGAPGQRVIISCSGSSSNVGSNTVNWYQQLPGTAPKLLIYDKNERPSGVPDRFSASKSGTSSSLAIGGLRSEDEADYYCATWDDNLNGWVFGGGTKLTVLG

SEQ ID NO: 298 - protein, 111 aa, Artificial Sequence
  clone 49m light chain
QSVLTQPPSASGAPGQRVIISCSGSSSNVGSNTVNWYQQLPGTAPKLLIYDKNERPSGVPDRFSASKSGTSSSLAIGGLRSEDEADYYCATWDDNLNGWVFGGGTKLTVLG

SEQ ID NO: 299 - protein, 124 aa, Artificial Sequence; identical to SEQ ID NO: 265
  clone 50 heavy chain

SEQ ID NO: 300 - protein, 111 aa, Artificial Sequence; identical to SEQ ID NO: 297
  clone 50 light chain

SEQ ID NO: 301 - protein, 111 aa, Artificial Sequence
  clone 50m light chain
QSVLTQPPSASGAPGQRVIISCSGSSSNVGSNTVNWYQQLPGTAPKLLIYDKNERPSGVPDRFSASKSGTSSSLAIGGLRSEDEADYYCGTWDDNLNGWVFGGGTKLTVLG

SEQ ID NO: 302 - protein, 124 aa, Artificial Sequence
  clone 51 heavy chain
EVQLVESGTEVKKPGASVKVSCKASGYTFTDYGLSWVRQAPGHGLEWMGWITAYNGDTNYAQKFQDRLSVTTDISTSTAYMELRSLKSDDTAVYYCARHVFCSGDGCYSGLGSWGQGTLVTVSS

SEQ ID NO: 303 - protein, 124 aa, Artificial Sequence
  clone 51m heavy chain
EVQLVQSGAEVKKPGASVKVSCKASGYTFTDYGLSWVRQAPGHGLEWMGWITAYNGDTNYAQKFQDRLSVTTDISTSTAYMELRSLKSDDTAVYYCARHVFCSGDGCYSGLGSWGQGTLVTVSS

SEQ ID NO: 304 - protein, 111 aa, Artificial Sequence; identical to SEQ ID NO: 301
  clone 51 light chain

SEQ ID NO: 305 - protein, 128 aa, Artificial Sequence
  clone 52 heavy chain
QVQLVQSGGGLVQPGGSLRISCTASGFTFRNYEMNWVRQAPGKGLEWVAYISSSGSSRYYADSVKGRFTISRDNAKNSLFLQMNSLRAEDMAVYYCARTDDGSSWFVSTSSFYGMDVWGQGTTVTVSS

SEQ ID NO: 306 - protein, 129 aa, Artificial Sequence
  clone 52m heavy chain
EQVQLVESGGGLVQPGGSLRISCTASGFTFRNYEMNWVRQAPGKGLEWVAYISSSGSSRYYADSVKGRFTISRDNAKNSLFLQMNSLRAEDMAVYYCARTDDGSSWFVSTSSFYGMDVWGQGTTVTVSS

SEQ ID NO: 307 - protein, 110 aa, Artificial Sequence
  clone 52 light chain
EIVLTQSPGIQSLSPGETATLSCRASESISSSYFAWYQQKPGQAPRLLIYGASSRASGIPDRFSGSGSGTDFTLTISRLEPEDFAVYYCQQYGSSPPITFGQGTRLEIKR

SEQ ID NO: 308 - protein, 128 aa, Artificial Sequence
  clone 53 heavy chain
QVQLVQSGGGLVQPGGSLRISCTASGFTFRNYEMNWVRQAPGKGLEWVAYISSSGSSRYYADSVKGRFTISRDNAKNTLYLQMSSLRSDDTAVYYCARTDDGSSWFVSTSSFYGMDVWGQGTTVTVSS

SEQ ID NO: 309 - protein, 129 aa, Artificial Sequence
  clone 53m heavy chain
EQVQLVESGGGLVQPGGSLRISCTASGFTFRNYEMNWVRQAPGKGLEWVAYISSSGSSRYYADSVKGRFTISRDNAKNTLYLQMSSLRSDDTAVYYCARTDDGSSWFVSTSSFYGMDVWGQGTTVTVSS

SEQ ID NO: 310 - protein, 110 aa, Artificial Sequence
  clone 53 light chain
DVVMTQSPGTLSLSPGERATLSCRASQSVSSSYLAWYQQKPGQAPRLLIYGVSSRATGIPDRFSGSGSGTDFTLTISRLEPEDFAVYYCQQYGSSPPITFGQGTKLEIKR

SEQ ID NO: 311 - protein, 110 aa, Artificial Sequence
  clone 53m light chain
EIVLTQSPGTLSLSPGERATLSCRASQSVSSSYLAWYQQKPGQAPRLLIYGVSSRATGIPDRFSGSGSGTDFTLTISRLEPEDFAVYYCQQYGSSPPITFGQGTKLEIKR

SEQ ID NO: 312 - protein, 120 aa, Artificial Sequence
  clone 54 heavy chain
EVQLVESGGGLVQPGGSLRLSCAASEFTFSMNWVRQAPGKGLEWVSSVRGGGTETYYADSVKGRFTVSRDNSKNTLYLQMNSLRVEDTAVYYCTVCVVMFRGWCNWFDPWGQGTLVTVSS

SEQ ID NO: 313 - protein, 108 aa, Artificial Sequence
  clone 54 light chain
DIQLTQSPSSVSASVGERVTITRRASQNIDRWLAWYQQKPGKAPDLLIFAASSLQSGVPSRFSGSGSGTDFTLTISSLQPEDFATYYCQQGKTFPPTFGQGTKLEIKR

SEQ ID NO: 314 - protein, 120 aa, Artificial Sequence
  clone 55 heavy chain
EVQLLESGGGLVQPGGSLRLSCAASEFTFSMNWVRQAPGKGLEWVSSVRGGGTETYYADSVKGRFTVSRDNSKNTLYLQMNSLRVEDTAVYYCTVCVVMFRGWCNWFDPWGQGTLVTVSS

SEQ ID NO: 315 - protein, 108 aa, Artificial Sequence
  clone 55 light chain
DVVMTQSPSSLSASVGDRVTITCRASQSLSSYLNWYQQKPGKAPKLLIYATTNLQSGVPSRFSGSGSGTHFTLTIGSLQPEDFATYYCQQSFQTPLTFGGGTKVEIKR

SEQ ID NO: 316 - protein, 108 aa, Artificial Sequence
  clone 55m light chain
DIQMTQSPSSLSASVGDRVTITCRASQSLSSYLNWYQQKPGKAPKLLIYATTNLQSGVPSRFSGSGSGTHFTLTIGSLQPEDFATYYCQQSFQTPLTFGGGTKLEIKR

SEQ ID NO: 317 - protein, 118 aa, Artificial Sequence
  clone 56 heavy chain
QVQLVESGGGVVQPGRSLRLSCAASGFTFISYVMHWVRQAPGKGLEWVAVVSYDGSEKYYADSVKGRFTISRDNSKNTLYLQMNSLTAEDTAVYYCAREPWVGTIDYWGQGTLVTVSS

SEQ ID NO: 318 - protein, 108 aa, Artificial Sequence
  clone 56 light chain
DIQMTQSPATLSASVGDRVTITCRASQSINNNLNWYQQKPGQAPKLLIYAASTLQGGVPSRFSGSGSGTEFTLTISSLQPEDFATYYCQQLNGYPLTFGGGTKVEIKR

SEQ ID NO: 319 - protein, 121 aa, Artificial Sequence
  clone 57 heavy chain
EVQLLESGGGLVQPGGSLRLSCAASGFTFSDYAMSWVRQAPGKGLEWVSSITANGLMTYYTDSVKGRFTISRDNSKNTLYLQMSSLRTDDTAVYYCAKDAGWEAWWYFDLWGRGTLVTVSS

SEQ ID NO: 320 - protein, 113 aa, Artificial Sequence
  clone 57 light chain
DIQMTQSPDSLAVSLGERATINCKSSQSVLYSSNNKNYLAWYQQKPGQPPKMLIYWASIRETGVPDRFSGSGSETDFTLTISSLQAEDVAVYYCQQYYSTLTFGGGTKVEIKR

SEQ ID NO: 321 - protein, 128 aa, Artificial Sequence
  clone 58 heavy chain
QVQLVQSGAEVKKPGASVKVSCKASGYTFTSYYMRWLRQAPGQGLEWMGIIDPSGGSTTYAQKFQGRVSITRDTSTSTVYMELSSLRSEDTAVYYCARGRGVVPAGNPSTGGVGMDVWGQGTTVTVSS

SEQ ID NO: 322 - protein, 108 aa, Artificial Sequence
  clone 58 light chain
EIVLTQSPATVSLSPGERTMLSCRASQNVSNYLGWYQQRRGQPPRLLISDASNRASGVPARFSGSGSGTDFTLTITSLQPEDFAVYFCQHRSSWPVTFGGGTKVEIKR

SEQ ID NO: 323 - protein, 122 aa, Artificial Sequence
  clone 59 heavy chain
QVQLVQSGSEVKKPGASVKVSCKASGYTFGHYGISWVRQAPGQGLEWMAWISAYNGNTDSIQKVQGRVTMTTDTSTNTAYLELRSLRSDDTAVYYCVRDVPATGGAATADYWGQGTLVTVSS

SEQ ID NO: 324 - protein, 113 aa, Artificial Sequence
  clone 59 light chain
DVVMTQSPLSLPVTLGQPASISCRSSQSLVFSDGNTYLSWFQQRPGQSPRRLIYKVSNRDSGVPDRFSASGSGTDFTLKISRVEADDVGVYYCMQVTHWPRTFGQGTKLEIKR

SEQ ID NO: 325 - protein, 122 aa, Artificial Sequence
  clone 60 heavy chain
QVQLVQSGPEVKKPGSSVKVSCKASGYTFGHYGISWVRQAPGQGLEWMAWISAYNGNTDSIQKVQGRVTMTTDTSTNTAYLELRSLRSDDTAVYYCVRDVPATGGAATADYWGQGTTVTVSS

SEQ ID NO: 326 - protein, 113 aa, Artificial Sequence
  clone 60 light chain
DVVMTQSPLSLPVTLGQPASISCRSSQSLVFSDGNTYLSWFQQRPGQSPRRLIYKVSNRDSGVPDRFSASGSGTDFTLKISRVEADDVGVYYCMQVTHWPRTFGQGTRLEIKR

SEQ ID NO: 327 - protein, 122 aa, Artificial Sequence
  clone 61 heavy chain
QVQLVQSGSEVKKPGASVKVSCKASGYTFGHYGISWVRQAPGQGLEWMAWISAYNGNTDSIQKVQGRVTMTTDTSTNTAYLELRSLRSDDTAVYYCVRDVPATGGAATADYWGQGTTVTVSS

SEQ ID NO: 328 - protein, 113 aa, Artificial Sequence; identical to SEQ ID NO: 324
  clone 61 light chain

SEQ ID NO: 329 - protein, 122 aa, Artificial Sequence
  clone 62 heavy chain
QVQLQQSGSEVKKPGASVKVSCKASGYTFGHYGISWVRQAPGQGLEWMAWISAYNGNTDSIQKVQGRVTMTTDTSTNTAYLELRSLRSDDTAVYYCVRDVPATGGAATADYWGQGTLVTVSS

SEQ ID NO: 330 - protein, 122 aa, Artificial Sequence
  clone 62m heavy chain
QVQLVQSGAEVKKPGASVKVSCKASGYTFGHYGISWVRQAPGQGLEWMAWISAYNGNTDSIQKVQGRVTMTTDTSTNTAYLELRSLRSDDTAVYYCVRDVPATGGAATADYWGQGTLVTVSS

SEQ ID NO: 331 - protein, 113 aa, Artificial Sequence
  clone 62 light chain
DVVMTQSPLSLPVPLGQPASISCRSSQSLVHSDGNTYLSWFQQRPGQSPRRLIYKVSDRDSGVPDRFSGSGSGTDFTLKISRVEAEDVGVYYCMQVTHWPRTFGQGTRLEIKR

SEQ ID NO: 332 - protein, 122 aa, Artificial Sequence; identical to SEQ ID NO: 323
  clone 63 heavy chain

SEQ ID NO: 333 - protein, 113 aa, Artificial Sequence
  clone 63 light chain
DVVMTQSPLSLPVTLGQPASISCKSSRSLVHSDGNTYLSWFQQRPGQSPRRLIYKVSNRDSGVPDRFSASGSGTDFTLKISRVEADDVGVYYCMQVTHWPRTFGQGTKLEIKR

SEQ ID NO: 334 - DNA, 18 bp, Artificial Sequence
  RT-IgGKLA primer
gtgtgcacgccgctggtc

SEQ ID NO: 335 - DNA, 22 bp, Artificial Sequence
  RT-IgGKLA primer
gtgggaagtttctggcggtcac

SEQ ID NO: 336 - DNA, 22 bp, Artificial Sequence
  RT-IgGKLA primer
tggagggcgttatccaccttcc

SEQ ID NO: 337 - DNA, 21 bp, Artificial Sequence
  RT-IgGKLA primer
gtgctcccttcatgcgtgacc

SEQ ID NO: 338 - DNA, 19 bp, Artificial Sequence
  primer_1st For
ccatggactggacctggag

SEQ ID NO: 339 - DNA, 24 bp, Artificial Sequence
  primer_1st For
gcttcctcctcctttggatctctg

SEQ ID NO: 340 - DNA, 21 bp, Artificial Sequence
  primer_1st For
atggacatactttgttccacg

SEQ ID NO: 341 - DNA, 17 bp, Artificial Sequence
  primer_1st For
ctsctgctctgggytcc

SEQ ID NO: 342 - DNA, 21 bp, Artificial Sequence
  primer_1st For
atggagtttgggctgagctgg

SEQ ID NO: 343 - DNA, 17 bp, Artificial Sequence
  primer_1st For
gtcctgggcccagtctg

SEQ ID NO: 344 - DNA, 20 bp, Artificial Sequence
  primer_1st For
atggaattggggctgagctg

SEQ ID NO: 345 - DNA, 20 bp, Artificial Sequence
  primer_1st For
cctgggctctgctsctcctc

SEQ ID NO: 346 - DNA, 20 bp, Artificial Sequence
  primer_1st For
atggagttgggactgagctg

SEQ ID NO: 347 - DNA, 23 bp, Artificial Sequence
  primer_1st For
gttctgtggtttcttctgagctg

SEQ ID NO: 348 - DNA, 17 bp, Artificial Sequence
  primer_1st For
atggaactggggctccg

SEQ ID NO: 349 - DNA, 20 bp, Artificial Sequence
  primer_1st For
gtggcctcctatgwgctgac

SEQ ID NO: 350 - DNA, 22 bp, Artificial Sequence
  primer_1st For
atgaaacacctgtggttcttcc

SEQ ID NO: 351 - DNA, 18 bp, Artificial Sequence
  primer_1st For
acagggtctctctcccag

SEQ ID NO: 352 - DNA, 18 bp, Artificial Sequence
  primer_1st For
atggggtcaaccgccatc

SEQ ID NO: 353 - DNA, 19 bp, Artificial Sequence
  primer_1st For
acaggtctctgtgctctgc

SEQ ID NO: 354 - DNA, 17 bp, Artificial Sequence
  primer_1st For
atgcaagtgggggcctc

SEQ ID NO: 355 - DNA, 19 bp, Artificial Sequence
  primer_1st For
attcycagrctgtggtgac

SEQ ID NO: 356 - DNA, 21 bp, Artificial Sequence
  primer_1st For
atgtctgtctccttcctcatc

SEQ ID NO: 357 - DNA, 21 bp, Artificial Sequence
  primer_1st For
gctcactgcacaggttcttgg

SEQ ID NO: 358 - DNA, 17 bp, Artificial Sequence
  primer_1st For
gctcagctcctggggct

SEQ ID NO: 359 - DNA, 18 bp, Artificial Sequence
  primer_1st For
tccctctcscagsctgtg

SEQ ID NO: 360 - DNA, 22 bp, Artificial Sequence
  primer_1st For
cttcctcctgctactctggctc

SEQ ID NO: 361 - DNA, 17 bp, Artificial Sequence
  primer_1st For
cagtggtccaggcaggg

SEQ ID NO: 362 - DNA, 24 bp, Artificial Sequence
  primer_1st For
tttctctgttgctctggatctctg

SEQ ID NO: 363 - DNA, 19 bp, Artificial Sequence
  primer_1st Rev
gcctgagttccacgacacc

SEQ ID NO: 364 - DNA, 25 bp, Artificial Sequence
  primer_1st Rev
ctgtactttggcctctctgggatag

SEQ ID NO: 365 - DNA, 19 bp, Artificial Sequence
  primer_1st Rev
ctgtccgctttcgctccag

SEQ ID NO: 366 - DNA, 20 bp, Artificial Sequence
  primer_1st Rev
ttccactgctcrggcgtcag

SEQ ID NO: 367 - DNA, 23 bp, Artificial Sequence
  primer_Nested For (VH)
caggtscagctggtgcagtctgg

SEQ ID NO: 368 - DNA, 22 bp, Artificial Sequence
  primer_Nested For (VH)
caggtgcagctgcaggagtcgg

SEQ ID NO: 369 - DNA, 26 bp, Artificial Sequence
  primer_Nested For (VH)
caggtcaccttgaaggagtctggtcc

SEQ ID NO: 370 - DNA, 22 bp, Artificial Sequence
  primer_Nested For (VH)
caggtgcagctacagcagtggg

SEQ ID NO: 371 - DNA, 23 bp, Artificial Sequence
  primer_Nested For (VH)
gaggtgcagctggtggagtctgg

SEQ ID NO: 372 - DNA, 23 bp, Artificial Sequence
  primer_Nested For (VH)
gargtgcagctggtgcagtctgg

SEQ ID NO: 373 - DNA, 23 bp, Artificial Sequence
  primer_Nested For (VH)
gaggtgcagctgttggagtctgg

SEQ ID NO: 374 - DNA, 23 bp, Artificial Sequence
  primer_Nested For (VH)
caggtacagctgcagcagtcagg

SEQ ID NO: 375 - DNA, 20 bp, Artificial Sequence
  primer_Nested For (VL)
cagtctgtgytgackcagcc

SEQ ID NO: 376 - DNA, 19 bp, Artificial Sequence
  primer_Nested For (VL)
caggcagggctgactcagc

SEQ ID NO: 377 - DNA, 20 bp, Artificial Sequence
  primer_Nested For (VL)
cagtctgccctgactcagcc

SEQ ID NO: 378 - DNA, 23 bp, Artificial Sequence
  primer_Nested For (VL)
gacatccagwtgacccagtctcc

SEQ ID NO: 379 - DNA, 21 bp, Artificial Sequence
  primer_Nested For (VL)
tcctatgagctgacwcagcca

SEQ ID NO: 380 - DNA, 27 bp, Artificial Sequence
  primer_Nested For (VL)
gatattgtgatgacccagwctccactc

SEQ ID NO: 381 - DNA, 22 bp, Artificial Sequence
  primer_Nested For (VL)
tcttctgagctgactcaggacc

SEQ ID NO: 382 - DNA, 25 bp, Artificial Sequence
  primer_Nested For (VL)
gaaattgtgttgacrcagtctccag

SEQ ID NO: 383 - DNA, 20 bp, Artificial Sequence
  primer_Nested For (VL)
cagcytgtgctgactcaatc

SEQ ID NO: 384 - DNA, 23 bp, Artificial Sequence
  primer_Nested For (VL)
gacatcgtgatgacccagtctcc

SEQ ID NO: 385 - DNA, 20 bp, Artificial Sequence
  primer_Nested For (VL)
cwgsctgtgctgactcagcc

SEQ ID NO: 386 - DNA, 23 bp, Artificial Sequence
  primer_Nested For (VL)
gaaacgacactcacgcagtctcc

SEQ ID NO: 387 - DNA, 24 bp, Artificial Sequence
  primer_Nested For (VL)
aattttatgctgactcagccccac

SEQ ID NO: 388 - DNA, 25 bp, Artificial Sequence
  primer_Nested For (VL)
gaaattgtgctgacwcagtctccag

SEQ ID NO: 389 - DNA, 21 bp, Artificial Sequence
  primer_Nested For (VL)
cagrctgtggtgacycaggag

SEQ ID NO: 390 - DNA, 22 bp, Artificial Sequence
  primer_Nested For (VL)
gacattgtgctgacccagtctc

SEQ ID NO: 391 - DNA, 22 bp, Artificial Sequence
  primer_Nested Rev
gggaagtagtccttgaccaggc

SEQ ID NO: 392 - DNA, 23 bp, Artificial Sequence
  primer_Nested Rev
gcacacaacagaggcagttccag

SEQ ID NO: 393 - DNA, 20 bp, Artificial Sequence
  primer_Nested Rev
tcacactgagtggctcctgg

SEQ ID NO: 394 - DNA, 23 bp, Artificial Sequence
  primer_Nested Rev
tgctggccgcrtacttgttgttg

SEQ ID NO: 395 - DNA, 38 bp, Artificial Sequence
  primer_VH For
ccgtggcccaggcggcccaggtgcagctggtgcagtct

SEQ ID NO: 396 - DNA, 38 bp, Artificial Sequence
  primer_VH For
ccgtggcccaggcggcccaggtgcagctggtggagtct

SEQ ID NO: 397 - DNA, 38 bp, Artificial Sequence
  primer_VH For
ccgtggcccaggcggcccaggtycagctkgtgcagtct

SEQ ID NO: 398 - DNA, 38 bp, Artificial Sequence
  primer_VH For
ccgtggcccaggcggccgaggtacagctcgtggagtcc

SEQ ID NO: 399 - DNA, 38 bp, Artificial Sequence
  primer_VH For
ccgtggcccaggcggcccaggttcagctggtgcagtct

SEQ ID NO: 400 - DNA, 37 bp, Artificial Sequence
  primer_VH For
ccgtggcccaggcggccaggtggagctgatagagtcc

SEQ ID NO: 401 - DNA, 38 bp, Artificial Sequence
  primer_VH For
ccgtggcccaggcggcccaggtccagctggtacagtct

SEQ ID NO: 402 - DNA, 38 bp, Artificial Sequence
  primer_VH For
ccgtggcccaggcggcccaggtrcagctggtggagtct

SEQ ID NO: 403 - DNA, 38 bp, Artificial Sequence
  primer_VH For
ccgtggcccaggcggcccaggtccagctggtgcagtct

SEQ ID NO: 404 - DNA, 38 bp, Artificial Sequence
  primer_VH For
ccgtggcccaggcggccgaggatcagctggtggagtct

SEQ ID NO: 405 - DNA, 38 bp, Artificial Sequence
  primer_VH For
ccgtggcccaggcggcccagatgcagctggtgcagtct

SEQ ID NO: 406 - DNA, 38 bp, Artificial Sequence
  primer_VH For
ccgtggcccaggcggccgaggtgcagctggtggagwct

SEQ ID NO: 407 - DNA, 38 bp, Artificial Sequence
  primer_VH For
ccgtggcccaggcggcccaaatgcagctggtgcagtct

SEQ ID NO: 408 - DNA, 38 bp, Artificial Sequence
  primer_VH For
ccgtggcccaggcggccsaggtgcagctggtggagtct

SEQ ID NO: 409 - DNA, 38 bp, Artificial Sequence
  primer_VH For
ccgtggcccaggcggccgaggtccagctggtacagtct

SEQ ID NO: 410 - DNA, 38 bp, Artificial Sequence
  primer_VH For
ccgtggcccaggcggccgaggtgcagctggtggagtcy

SEQ ID NO: 411 - DNA, 38 bp, Artificial Sequence
  primer_VH For
ccgtggcccaggcggcccagrtcaccttgaaggagtct

SEQ ID NO: 412 - DNA, 38 bp, Artificial Sequence
  primer_VH For
ccgtggcccaggcggcccaggtgcagctgcaggagtyg

SEQ ID NO: 413 - DNA, 38 bp, Artificial Sequence
  primer_VH For
ccgtggcccaggcggcccaggtcaccttgaaggagtct

SEQ ID NO: 414 - DNA, 38 bp, Artificial Sequence
  primer_VH For
ccgtggcccaggcggcccaggtgcagctgcaggagtcg

SEQ ID NO: 415 - DNA, 38 bp, Artificial Sequence
  primer_VH For
ccgtggcccaggcggcccaggtcaccttgarggagtct

SEQ ID NO: 416 - DNA, 38 bp, Artificial Sequence
  primer_VH For
ccgtggcccaggcggcccagctgcagctgcaggagtcc

SEQ ID NO: 417 - DNA, 38 bp, Artificial Sequence
  primer_VH For
ccgtggcccaggcggccgaggtgcagctggtggagtct

SEQ ID NO: 418 - DNA, 38 bp, Artificial Sequence
  primer_VH For
ccgtggcccaggcggcccaggtgcagctgcaggastcg

SEQ ID NO: 419 - DNA, 38 bp, Artificial Sequence
  primer_VH For
ccgtggcccaggcggccgaagtgcagctggtggagtct

SEQ ID NO: 420 - DNA, 38 bp, Artificial Sequence
  primer_VH For
ccgtggcccaggcggcccaggtgcrgctgcaggagtcg

SEQ ID NO: 421 - DNA, 38 bp, Artificial Sequence
  primer_VH For
ccgtggcccaggcggcccaggtgcagctgktggagtct

SEQ ID NO: 422 - DNA, 38 bp, Artificial Sequence
  primer_VH For
ccgtggcccaggcggcccaggtgcagctrcarsagtsg

SEQ ID NO: 423 - DNA, 38 bp, Artificial Sequence
  primer_VH For
ccgtggcccaggcggccgaggtgcakctggtggagtct

SEQ ID NO: 424 - DNA, 38 bp, Artificial Sequence
  primer_VH For
ccgtggcccaggcggcccagstgcagctgcaggagtcg

SEQ ID NO: 425 - DNA, 38 bp, Artificial Sequence
  primer_VH For
ccgtggcccaggcggccgaggtrcarctggtggagtct

SEQ ID NO: 426 - DNA, 38 bp, Artificial Sequence
  primer_VH For
ccgtggcccaggcggccgaagtgcagctggtgcagtcy

SEQ ID NO: 427 - DNA, 38 bp, Artificial Sequence
  primer_VH For
ccgtggcccaggcggccacagtgcagctggtggagtct

SEQ ID NO: 428 - DNA, 38 bp, Artificial Sequence
  primer_VH For
ccgtggcccaggcggccgaggtgcagctggtgcagtct

SEQ ID NO: 429 - DNA, 38 bp, Artificial Sequence
  primer_VH For
ccgtggcccaggcggccgaggtgcarctggtggagtct

SEQ ID NO: 430 - DNA, 38 bp, Artificial Sequence
  primer_VH For
ccgtggcccaggcggcccaggtacagctgcagcagtca

SEQ ID NO: 431 - DNA, 38 bp, Artificial Sequence
  primer_VH For
ccgtggcccaggcggccgaggtgcagctgktggagtct

SEQ ID NO: 432 - DNA, 38 bp, Artificial Sequence
  primer_VH For
ccgtggcccaggcggcccaggtgcagctggtgcaatct

SEQ ID NO: 433 - DNA, 38 bp, Artificial Sequence
  primer_VH For
ccgtggcccaggcggccgagaygcagctggtggagtct

SEQ ID NO: 434 - DNA, 38 bp, Artificial Sequence
  primer_VH For
ccgtggcccaggcggccctgcagctggtgcagtctggg

SEQ ID NO: 435 - DNA, 38 bp, Artificial Sequence
  primer_VH For
ccgtggcccaggcggccgaggtggagctgatagagccc

SEQ ID NO: 436 - DNA, 38 bp, Artificial Sequence; identical to SEQ ID NO: 395
  primer_VH For

SEQ ID NO: 437 - DNA, 55 bp, Artificial Sequence
  primer_JH Rev
gcctgaaccacctccgccagatccgccacctcctgaggagacggtgaccagggtg

SEQ ID NO: 438 - DNA, 54 bp, Artificial Sequence
  primer_JH Rev
gcctgaaccacctccgccagatccgccacctcctgaggagacggtgaccagggt

SEQ ID NO: 439 - DNA, 56 bp, Artificial Sequence
  primer_JH Rev
gcctgaaccacctccgccagatccgccacctcctgaggagacagtgaccagggtgc

SEQ ID NO: 440 - DNA, 55 bp, Artificial Sequence
  primer_JH Rev
gcctgaaccacctccgccagatccgccacctcctgaggagacggtgaccgtggtc

SEQ ID NO: 441 - DNA, 57 bp, Artificial Sequence
  primer_JH Rev
tctggcggaggtggttcaggcggtggaggctcggacatccagatgacccagtctcct

SEQ ID NO: 442 - DNA, 57 bp, Artificial Sequence; identical to SEQ ID NO: 441
  primer_V kappa For

SEQ ID NO: 443 - DNA, 57 bp, Artificial Sequence
  primer_V kappa For
tctggcggaggtggttcaggcggtggaggctcggatgttgtgatgactcagtctcca

SEQ ID NO: 444 - DNA, 57 bp, Artificial Sequence
  primer_V kappa For
tctggcggaggtggttcaggcggtggaggctcggccatccagatgacccagtctcca

SEQ ID NO: 445 - DNA, 57 bp, Artificial Sequence
  primer_V kappa For
tctggcggaggtggttcaggcggtggaggctcggagattgtgatgacccagactcca

SEQ ID NO: 446 - DNA, 57 bp, Artificial Sequence
  primer_V kappa For
tctggcggaggtggttcaggcggtggaggctcggycatcyggatgacccagtctcca

SEQ ID NO: 447 - DNA, 57 bp, Artificial Sequence
  primer_V kappa For
tctggcggaggtggttcaggcggtggaggctcggaaattgtaatgacacagtctcaa

SEQ ID NO: 448 - DNA, 57 bp, Artificial Sequence
  primer_V kappa For
tctggcggaggtggttcaggcggtggaggctcggacatccagttgacccagtctcca

SEQ ID NO: 449 - DNA, 57 bp, Artificial Sequence
  primer_V kappa For
tctggcggaggtggttcaggcggtggaggctcggaaattgtgttgacacagtctcca

SEQ ID NO: 450 - DNA, 57 bp, Artificial Sequence
  primer_V kappa For
tctggcggaggtggttcaggcggtggaggctcggacatccagatgacccagtctcca

SEQ ID NO: 451 - DNA, 57 bp, Artificial Sequence
  primer_V kappa For
tctggcggaggtggttcaggcggtggaggctcggaaatagtgatgasgcagtctcca

SEQ ID NO: 452 - DNA, 57 bp, Artificial Sequence
  primer_V kappa For
tctggcggaggtggttcaggcggtggaggctcggccatccagttgacccagtctcca

SEQ ID NO: 453 - DNA, 57 bp, Artificial Sequence
  primer_V kappa For
tctggcggaggtggttcaggcggtggaggctcggaaattgtgttgacrcagtctcca

SEQ ID NO: 454 - DNA, 57 bp, Artificial Sequence
  primer_V kappa For
tctggcggaggtggttcaggcggtggaggctcgracatccagatgacccagtctcca

SEQ ID NO: 455 - DNA, 57 bp, Artificial Sequence
  primer_V kappa For
tctggcggaggtggttcaggcggtggaggctcggacatcgtgatgacccagtctcca

SEQ ID NO: 456 - DNA, 57 bp, Artificial Sequence
  primer_V kappa For
tctggcggaggtggttcaggcggtggaggctcggacatccagatgayccagtctcca

SEQ ID NO: 457 - DNA, 57 bp, Artificial Sequence
  primer_V kappa For
tctggcggaggtggttcaggcggtggaggctcggaaacgacactcacgcagtctcca

SEQ ID NO: 458 - DNA, 57 bp, Artificial Sequence; identical to SEQ ID NO: 456
  primer_V kappa For

SEQ ID NO: 459 - DNA, 57 bp, Artificial Sequence
  primer_V kappa For
tctggcggaggtggttcaggcggtggaggctcggaaattgtgctgactcagtctcca

SEQ ID NO: 460 - DNA, 57 bp, Artificial Sequence
  primer_V kappa For
tctggcggaggtggttcaggcggtggaggctcggatattgtgatgacccagcatctg

SEQ ID NO: 461 - DNA, 57 bp, Artificial Sequence
  primer_V kappa For
tctggcggaggtggttcaggcggtggaggctcggatgttgtgatgacacagtctcca

SEQ ID NO: 462 - DNA, 57 bp, Artificial Sequence
  primer_V kappa For
tctggcggaggtggttcaggcggtggaggctcggatattgtgatgacccagactcca

SEQ ID NO: 463 - DNA, 57 bp, Artificial Sequence
  primer_V kappa For
tctggcggaggtggttcaggcggtggaggctcggacattgtgctgacccagtctcca

SEQ ID NO: 464 - DNA, 57 bp, Artificial Sequence
  primer_V kappa For
tctggcggaggtggttcaggcggtggaggctcggatattgtgatgactcagtctcca

SEQ ID NO: 465 - DNA, 44 bp, Artificial Sequence
  primer_J kappa Rev
tgctggccggcctggcctcgtttgatctccagcttggtcccctg

SEQ ID NO: 466 - DNA, 44 bp, Artificial Sequence
  primer_J kappa Rev
tgctggccggcctggcctcgtttgatctccaccttggtccctcc

SEQ ID NO: 467 - DNA, 47 bp, Artificial Sequence
  primer_J kappa Rev
tgctggccggcctggcctcgtttgatatccactttggtcccagggcc

SEQ ID NO: 468 - DNA, 47 bp, Artificial Sequence
  primer_V kappa For
tgctggccggcctggcctcgtttaatctccagtcgtgtcccttggcc

SEQ ID NO: 469 - DNA, 56 bp, Artificial Sequence
  primer_V lambda For
tctggcggaggtggttcaggcggtggaggctcgcagtctgtgctgactcagccacc

SEQ ID NO: 470 - DNA, 56 bp, Artificial Sequence
  primer_V lambda For
tctggcggaggtggttcaggcggtggaggctcgcagtctgccctgactcagcctca

SEQ ID NO: 471 - DNA, 54 bp, Artificial Sequence
  primer_V lambda For
tctggcggaggtggttcaggcggtggaggctcgcagtctgtsstgacgcagccg

SEQ ID NO: 472 - DNA, 57 bp, Artificial Sequence
  primer_V lambda For
tctggcggaggtggttcaggcggtggaggctcgtcctatgagctgayrcagccaccc

SEQ ID NO: 473 - DNA, 55 bp, Artificial Sequence
  primer_V lambda For
tctggcggaggtggttcaggcggtggaggctcgcagtctgtgttgacgcagccgc

SEQ ID NO: 474 - DNA, 57 bp, Artificial Sequence
  primer_V lambda For
tctggcggaggtggttcaggcggtggaggctcgtcctccatgctgactcaggagcca

SEQ ID NO: 475 - DNA, 55 bp, Artificial Sequence
  primer_V lambda For
tctggcggaggtggttcaggcggtggaggctcgcagyctgtgctgactcagccac

SEQ ID NO: 476 - DNA, 59 bp, Artificial Sequence
  primer_V lambda For
tctggcggaggtggttcaggcggtggaggctcgtcctatgagctgacacagccaycctc

SEQ ID NO: 477 - DNA, 54 bp, Artificial Sequence
  primer_V lambda For
tctggcggaggtggttcaggcggtggaggctcgcagtctgtgytgacgcagccg

SEQ ID NO: 478 - DNA, 57 bp, Artificial Sequence
  primer_V lambda For
tctggcggaggtggttcaggcggtggaggctcgacatatgagctgtctcagccaccc

SEQ ID NO: 479 - DNA, 57 bp, Artificial Sequence
  primer_V lambda For
tctggcggaggtggttcaggcggtggaggctcgcagcctgtgctgactcagatgacc

SEQ ID NO: 480 - DNA, 57 bp, Artificial Sequence
  primer_V lambda For
tctggcggaggtggttcaggcggtggaggctcgtcctctgagctgagtcaggagcct

SEQ ID NO: 481 - DNA, 55 bp, Artificial Sequence
  primer_V lambda For
tctggcggaggtggttcaggcggtggaggctcgcagtctgccctgaytcagcctc

SEQ ID NO: 482 - DNA, 55 bp, Artificial Sequence
  primer_V lambda For
tctggcggaggtggttcaggcggtggaggctcgtcctctgggccaactcaggtgc

SEQ ID NO: 483 - DNA, 55 bp, Artificial Sequence
  primer_V lambda For
tctggcggaggtggttcaggcggtggaggctcgcartctgccctgactcagccts

SEQ ID NO: 484 - DNA, 54 bp, Artificial Sequence
  primer_V lambda For
tctggcggaggtggttcaggcggtggaggctcgctgcctgtgctgactcagccc

SEQ ID NO: 485 - DNA, 57 bp, Artificial Sequence
  primer_V lambda For
tctggcggaggtggttcaggcggtggaggctcgcagtctgttctgactcagcctcgc

SEQ ID NO: 486 - DNA, 57 bp, Artificial Sequence
  primer_V lambda For
tctggcggaggtggttcaggcggtggaggctcgcagcctgtgctgactcaatcatcc

SEQ ID NO: 487 - DNA, 57 bp, Artificial Sequence
  primer_V lambda For
tctggcggaggtggttcaggcggtggaggctcgtcctatgagctgactcagccaccc

SEQ ID NO: 488 - DNA, 57 bp, Artificial Sequence
  primer_V lambda For
tctggcggaggtggttcaggcggtggaggctcgcagcttgtgctgactcaatcgccc

SEQ ID NO: 489 - DNA, 57 bp, Artificial Sequence
  primer_V lambda For
tctggcggaggtggttcaggcggtggaggctcgtcctctgagctgactcagctgcct

SEQ ID NO: 490 - DNA, 54 bp, Artificial Sequence
  primer_V lambda For
tctggcggaggtggttcaggcggtggaggctcgcagcctgtgctgactcagccr

SEQ ID NO: 491 - DNA, 59 bp, Artificial Sequence
  primer_V lambda For
tctggcggaggtggttcaggcggtggaggctcgtcctatgagcttacacagccaccctc

SEQ ID NO: 492 - DNA, 60 bp, Artificial Sequence
  primer_V lambda For
tctggcggaggtggttcaggcggtggaggctcgaattttatgctgactcagccccactct

SEQ ID NO: 493 - DNA, 57 bp, Artificial Sequence
  primer_V lambda For
tctggcggaggtggttcaggcggtggaggctcgtcctctgagcggactcagttgcct

SEQ ID NO: 494 - DNA, 56 bp, Artificial Sequence
  primer_V lambda For
tctggcggaggtggttcaggcggtggaggctcgcagrctgtggtgactcaggagcc

SEQ ID NO: 495 - DNA, 59 bp, Artificial Sequence
  primer_V lambda For
tctggcggaggtggttcaggcggtggaggctcgtcctatgagctgactcagccactctc

SEQ ID NO: 496 - DNA, 54 bp, Artificial Sequence
  primer_V lambda For
tctggcggaggtggttcaggcggtggaggctcgcagactgtggtgacccaggag

SEQ ID NO: 497 - DNA, 57 bp, Artificial Sequence
  primer_V lambda For
tctggcggaggtggttcaggcggtggaggctcgtcctatgagctgacwcagccacmc

SEQ ID NO: 498 - DNA, 54 bp, Artificial Sequence
  primer_V lambda For
tctggcggaggtggttcaggcggtggaggctcgcagcctgtgctgactcagcca

SEQ ID NO: 499 - DNA, 58 bp, Artificial Sequence
  primer_V lambda For
tctggcggaggtggttcaggcggtggaggctcgtcttctgagctgactcaggaccctg

SEQ ID NO: 500 - DNA, 54 bp, Artificial Sequence
  primer_V lambda For
tctggcggaggtggttcaggcggtggaggctcgcaggcagggctgactcagcca

SEQ ID NO: 501 - DNA, 57 bp, Artificial Sequence
  primer_V lambda For
tctggcggaggtggttcaggcggtggaggctcgtcctatgtgctgacwcagcyaccc

SEQ ID NO: 502 - DNA, 51 bp, Artificial Sequence
  primer_V lambda For
tctggcggaggtggttcaggcggtggaggctcgcggcccgtgctgactcag

SEQ ID NO: 503 - DNA, 44 bp, Artificial Sequence
  primer_J lambda Rev
tgctggccggcctggccgcctaggacggtgaccttggtcccagt

SEQ ID NO: 504 - DNA, 41 bp, Artificial Sequence
  primer_J lambda Rev
tgctggccggcctggccgcctaggacggtcagctcsgtccc

SEQ ID NO: 505 - DNA, 43 bp, Artificial Sequence
  primer_J lambda Rev
tgctggccggcctggccgcctaggacggtcagcttggtccctc

SEQ ID NO: 506 - DNA, 42 bp, Artificial Sequence
  primer_J lambda Rev
tgctggccggcctggccgccgaggacggtcaccttggtgcca

SEQ ID NO: 507 - DNA, 52 bp, Artificial Sequence
  primer_J lambda Rev
tgctggccggcctggccgcctaaaatgatcagctgggttcctccaccaaata

SEQ ID NO: 508 - DNA, 40 bp, Artificial Sequence
  primer_J lambda Rev
tgctggccggcctggccgccgaggycggtcagctgggtgc

SEQ ID NO: 509 - DNA, 48 bp, Artificial Sequence
  IgG_primer_Heavy chain_HC_F1
tgctgtgggtgagtggtacctgtggggaggtgcagctggtggagtctg

SEQ ID NO: 510 - DNA, 50 bp, Artificial Sequence
  IgG_primer_Heavy chain_HC_F2
tgctgtgggtgagtggtacctgtgggcaggtcaccttgaaggagtctggg

SEQ ID NO: 511 - DNA, 48 bp, Artificial Sequence
  IgG_primer_Heavy chain_HC_F3
tgctgtgggtgagtggtacctgtgggcaggtgcagctggtgcagtctg

SEQ ID NO: 512 - DNA, 54 bp, Artificial Sequence
  IgG_primer_Heavy chain_HC_R1
gggggaagaccgatgggcccttggtggaggctgaggagacggtgaccagggttc

SEQ ID NO: 513 - DNA, 55 bp, Artificial Sequence
  IgG_primer_Heavy chain_HC_R2
gggggaagaccgatgggcccttggtggaggctgaggagacagtgaccagggttcc

SEQ ID NO: 514 - DNA, 54 bp, Artificial Sequence
  IgG_primer_Heavy chain_HC_R3
gggggaagaccgatgggcccttggtggaggctgaggagacggtgaccgtggttc

SEQ ID NO: 515 - DNA, 53 bp, Artificial Sequence
  IgG_primer_Heavy chain_HC_R4
gggggaagaccgatgggcccttggtggaggctgaggagacggtgaccgtggtc

SEQ ID NO: 516 - DNA, 47 bp, Artificial Sequence
  IgG_primer_Lambda chain_LC_F1
tgctgtgggtgagtggtacctgtgggcagtctgtgctgacgcagccg

SEQ ID NO: 517 - DNA, 48 bp, Artificial Sequence
  IgG_primer_Lambda chain_LC_F2
tgctgtgggtgagtggtacctgtgggtcctatgagctgactcagccac

SEQ ID NO: 518 - DNA, 48 bp, Artificial Sequence
  IgG_primer_Lambda chain_LC_F3
tgctgtgggtgagtggtacctgtgggcagcctgtgctgactcagccac

SEQ ID NO: 519 - DNA, 49 bp, Artificial Sequence
  IgG_primer_Lambda chain_LC_F4
tgctgtgggtgagtggtacctgtgggcagactgtggtgactcaggagcc

SEQ ID NO: 520 - DNA, 48 bp, Artificial Sequence
  IgG_primer_Lambda chain_LC_F5
tgctgtgggtgagtggtacctgtgggcagtctgccctgactcagcctg

SEQ ID NO: 521 - DNA, 42 bp, Artificial Sequence
  IgG_primer_Lambda chain_LC_R1
gtgggattggccttaggttggcctaggacggtgaccttggtc

SEQ ID NO: 522 - DNA, 42 bp, Artificial Sequence
  IgG_primer_Lambda chain_LC_R2
gtgggattggccttaggttggcctaggacggtcagcttggtc

SEQ ID NO: 523 - DNA, 50 bp, Artificial Sequence
  IgG_primer_Kappa chain_KC_F1
tgctgtgggtgagtggtacctgtggggatgttgtgatgactcagtctcca

SEQ ID NO: 524 - DNA, 50 bp, Artificial Sequence
  IgG_primer_Kappa chain_KC_F2
tgctgtgggtgagtggtacctgtggggatattgtgatgacccagactcca

SEQ ID NO: 525 - DNA, 50 bp, Artificial Sequence
  IgG_primer_Kappa chain_KC_F3
tgctgtgggtgagtggtacctgtggggacatccagatgacccagtctcca

SEQ ID NO: 526 - DNA, 50 bp, Artificial Sequence
  IgG_primer_Kappa chain_KC_F4
tgctgtgggtgagtggtacctgtggggagattgtgctgacccagtctcca

SEQ ID NO: 527 - DNA, 50 bp, Artificial Sequence
  IgG_primer_Kappa chain_KC_F5
tgctgtgggtgagtggtacctgtggggacatccagttgacccagtctcca

SEQ ID NO: 528 - DNA, 44 bp, Artificial Sequence
  IgG_primer_Kappa chain_KC_R1
acgcttggagcggccaccgtacgtttgatctccagcttggtccc

SEQ ID NO: 529 - DNA, 47 bp, Artificial Sequence
  IgG_primer_Kappa chain_KC_R2
acgcttggagcggccaccgtacgtttaatctccagtcgtgtcccttg

SEQ ID NO: 530 - DNA, 44 bp, Artificial Sequence
  IgG_primer_Kappa chain_KC_R3
acgcttggagcggccaccgtacgtttgatctccaccttggtccc